European Patent Application EP 4 516 907 A2, published March 5, 2025. Title: METHODS OF MAKING AND USING UNIVERSAL CENTRALIZED INFLUENZA VACCINE GENES. Applicant: Board of Regents of the University of Nebraska. The sequence listing filed with the application follows.

SEQUENCE LISTING (122 sequences)

SEQ ID NO: 1 - protein, 572 aa, synthetic construct
  REGION 1..572: note = synthetically-generated protein
MKAILVVLLYTFATANADTLCIGYHANNSTDTVDTVLEKNVTVTHSVNLLEDKHNGKLCKLRGVAPLHLGKCNIAGWILGNPECESLSTASSWSYIVETSSSDNGTCYPGDFIDYEELREQLSSVSSFERFEIFPKTSSWPNHDSNKGVTAACPHAGAKSFYKNLIWLVKKGNSYPKLSKSYINDKGKEVLVLWGIHHPSTADQQSLYQNADAYVFVGTSRYSKKFKPEIAIRPKVRDQEGRMNYYWTLVEPGDKITFEATGNLVVPRYAFAMERNAGSGIIISDTPVHDCNTTCQTPKGAINTSLTSLPFQNIHPITIGKCPKYVKSTKLRLATGLRNVPSIQSRGLFGAIAGFIEGGWTGMVDGWYGYHHQNEQGSGYAADLKSTQNAIDITNKVNSVIEKMNTQFTAVGKEFNHLEKRIENLNKKVDDGFLDIWTYNAELLVLLENERTLDYHDSNVKNLYEKVRSQLKNNAKEIGNGCFEFYHKCDNTCMESVKNGTYDYPKYSEEAKLNREEIDGVKLESTRIYQILAIYSTVASSLVLVVSLGAISFWMCSNGSSVEYSLQCRICI

SEQ ID NO: 2 - protein, 560 aa, synthetic construct
  REGION 1..560: note = synthetically-generated protein
MKVKLLVLLCTFTATYADTICIGYHANNSTDTVDTVLEKNVTVTHSVNLLEDSHNGKLCLLKGIAPLQLGNCSVAGWILGNPECELLISKESWSYIVETPNPENGTCYPGFADYEELREQLSSVSSFERFEIFPKESSWPNHTVTKGVSASCSHNGSSFYRNLLWLTGKNGLYPNLSKSYANNKEKEVLVLWGVHHPPNIGDQLYHTENAYVSVVSSHYSRFTPEIAKRPKVRDQEGRINYYWTLLEPGDTIIFEANGNLIAPRYAFALSRGFGSGIISNAPMDECDAKCQTPQGAINSSLPFQNVHPVTIGECPKYVRSAKLRMVTGLRNIPSIQSRGLFGAIAGFIEGGWTGMVDGWYGYHHQNEQGSGYAADQKSTQNAINGITNKVNSVIEKMNTQFTAVGKEFNKLERRMENLNKKVDDGFLDIWTYNAELLVLLENERTLDFHDSNVKNLYEKVKSQLKNNAKEIGNGCFEFYHKCNDECMESVKNGTYDYPKYSEESKLNREKIDGVKLESMGVYQILAIYSTVASSLVLLVSLGAISFWMCSNGSLQCRICI

SEQ ID NO: 3 - protein, 565 aa, synthetic construct
  REGION 1..565: note = synthetically-generated protein
MKVKLLVLLCTFTATYADTICIGYHANNSTDTVDTVLEKNVTVTHSVNLLENSHNGKLCLLKGIAPLQLGNCSVAGWILGNPECELLISKESWSYIVEKPNPENGTCYPGHFADYEELREQLSSVSSLERFEIFPKESSWPNHTVTGVSASCSHNGESSFYRNLLWLTGKNGLYPNLSKSYANNKEKEVLVLWGVHHPPNIGDQRALYHTENAYVSVVSSHYSRKFTPEIAKRPKVRDQEGRINYYWTLLEPGDTIIFEANGNLIAPRYAFALSRGFGSGIINSNAPMDKCDAKCQTPQGAINSSLPFQNVHPVTIGECPKYVRSAKLRMVTGLRNIPSVQSRGLFGAIAGFIEGGWTGMIDGWYGYHHQNEQGSGYAADQKSTQNAINGITNKVNSVIEKMNIQFTAVGKEFNKLERRMENLNKKVDDGFIDIWTYNAELLVLLENERTLDFHDSNVKNLYEKVKSQLKNNAKEVGNGCFEFYHKCNDECMESVKNETYDYPKYSEESKLNREKIDGVKLDSMGVYQILTIYSTVASSLVLLVSLGAISFWMCSNGSLQCKICI

SEQ ID NO: 4 - protein, 566 aa, synthetic construct
  REGION 1..566: note = synthetically-generated protein
MKAILVVLLYTFTTANADTLCIGYHANNSTDTVDTILEKNVTVTHSVNLLEDKHNGKLCKLRGVAPLHLGKCNIAGWILGNPECESLSTASSWSYIVETSNSDNGTCYPGDFINYEELREQLSSVSSFERFEIFPKTSSWPNHDPNKGVTTACPHAGAKSFYKNLIWLVEKGNSYPKLSKSYINDKGKEILVLWGIHHPSTSADQQSLYQNADTYVFVGTSKYSKKFKPEIAIRPKVRDQEGRMNYYWTLIEPGDKITFETTGNLVVPRYAFAMERNAGSGIIISDTSVHDCNTTCQTPKGAINTSLPFHNIHPITIGECPKYVRSTKLRMVTGLRNIPSIQSRGLFGAIAGFIEGGWTGMVDGWYGYHHQNAQGSGYAADQKSTQNAIDEITNKVNSVIEKMNTQFTAVGKEFNKLEKRMENLNKKVDDGFLDIWTYNAELLILLENERTLDYHDSNVKNLYEKVRSQLKNNAKETGNGCFEFYHKCDNTCMESVKNGTYNYPKYSEEAKLNREKIDGVKLESMGVYQILAIYSTVASSLVLVVSLGAVSFWMCSNGSLRCRICI

SEQ ID NO: 5 - protein, 566 aa, synthetic construct
  REGION 1..566: note = synthetically-generated protein
MEAILVVLLYTFATANADTLCVGYHANNSTDTVDTLLEKNVTVTHSVNLLEDSHNGKLCRLKGIAPLQLGKCSIAGWILGNPECETLSTASSWSYIVETSSSDNGTCYPGDFIDYEELREQLSSVSSFERFEMFPKTSSWPNHDSNKGVTAACPHAGAKGFYKNLIWLVKKGNSYPKLSQSYINDKGKEVLVLWGIHHPSTTADQQSLYQNADAYVFVGTSRYSKKFKPEIATRPKVRDQERRMNYYWTLVEPGDKITFEATGNLVVPRYAFTMERNAGSGIIISDTPVHDCNTTCQTPEGAINTSLPFQNIHPITIGKCPKYVKSTKLRLATGLRNVPSIQSRGLLGAIAGFIEGGWTGMMDGWYGYHHQNGQGSGYAADLKSTQNAIDKITNKVNSVIDKMNTQFTAVGKEFNHLEKRIENLNKKVDDGFIDVWTYNAELLVVLENERTLEYHDSNVKNLYEKVRNQLKNNAKEIGNGCFEFYHKCNNECMESVKNGTYDYPKYSEEAKLNREEIDGVKLESTRIYQILAIYSTAASSLVLVVSLGAISFWMCSNGSLQCRICI

SEQ ID NO: 6 - protein, 566 aa, synthetic construct
  REGION 1..566: note = synthetically-generated protein
MKAILVVLLYTFATANADTLCIGYHANNSTDTVDTVLEKNVTVTHSVNLLEDKHNGKLCKLRGVAPLHLGKCNIAGWILGNPECESLSTASSWSYIVETSSSDNGTCYPGDFIDYEELREQLSSVSSFERFEIFPKTSSWPNHDSNKGVTAACPHAGAKSFYKNLIWLVKKGNSYPKLSKSYINDKGKEVLVLWGIHHPSTSADQQSLYQNADAYVFVGTSRYSKKFKPEIAIRPKVRDQEGRMNYYWTLVEPGDKITFEATGNLVVPRYAFAMERNAGSGIIISDTPVHDCNTTCQTPKGAINTSLPFQNIHPITIGKCPKYVKSTKLRLATGLRNVPSIQSRGLFGAIAGFIEGGWTGMVDGWYGYHHQNEQGSGYAADLKSTQNAIDKITNKVNSVIEKMNTQFTAVGKEFNHLEKRIENLNKKVDDGFLDIWTYNAELLVLLENERTLDYHDSNVKNLYEKVRSQLKNNAKEIGNGCFEFYHKCDNTCMESVKNGTYDYPKYSEEAKLNREEIDGVKLESTRIYQILAIYSTVASSLVLVVSLGAISFWMCSNGSLQCRICI

SEQ ID NO: 7 - protein, 563 aa, synthetic construct
  REGION 1..563: note = synthetically-generated protein
MKVKLLVLLCTFTATYADTICIGYHANNSTDTVDTILEKNVTVTHSVNLLENSHNGKLCLLKGIAPLQLGNCSVAGWILGNPECELLISKESWSYIVEKPNPENGTCYPGDFINYEELREQLSSVSSLERFEIFPKESSWPNHTVTGVSASCSHNGESSFYRNLLWLTGKNGLYPNLSKSYANNKEKEVLVLWGVHHPPNIGDQRALYHTENAYVSVVSSHYSRKFTPEIAKRPKVRDQEGRINYYWTLLEPGDTIIFEANGNLIAPRYAFALSRGFGSGIINSNAPMDKCDAKCQTPQGAINSSLPFQNVHPVTIGECPKYVRSAKLRMVTGLRNIPSIQSRGLLGAIAGFIEGGWTGMIDGWYGYHHQNAQGSGYAADQKSTQNAIDEITNKVNSVIEKMNIQFTAVGKEFNKLERRMENLNKKVDDGFIDIWTYNAELLILLENERTLDFHDSNVKNLYEKVRNQLKNNAKEVGNGCFEFYHKCNDECMESVKNGIYDYPKYSEESKLNREKIDGVKLESMGVYQILAIYSTVASSLVLLVSLGAISFWMCSGHSCRICI

SEQ ID NO: 8 - protein, 566 aa, synthetic construct
  REGION 1..566: note = synthetically-generated protein
MEAILVVLLYTFTTANADTLCVGYHANNSTDTVDTVLERNVTVTHSVNLLEDSHNGKLCRLKGIAPLQLGKCNIAGWLLGNPECESLFSKESWSYIVETPNPENGTCYPGHFADYEELREQLNSVSSFERFEMFPKTSSWPDHDSNKGVTTACPHAGAKGFYKNLIWLTKKGNSYPKLSQSYINDKGKEILVLWGIHHPSTTADQQSLYQNADTYVFVGTSKYSKKFKPEIATRPKVRDQERRMNYYWTLIEPGDKITFEANGNLVVPRYAFTMERNAGSGIIISDTSVHDCNTTCQTPEGAINTSLPFHNIHPITIGECPKYVRSTKLRMVTGLRNVPSVQSRGLFGAIAGFIEGGWTGMMDGWYGYHHQNGQGSGYAADQKSTQNAINGITNKVNSVIDKMNTQFTAVGKEFNKLEKRMENLNKKVDDGFIDVWTYNAELLILLENERTLDYHDSKVKNLYEKVKSQLKNNAKETGNGCFEFYHKCNNECMESVKNGTYDYPRYSEEAKLNREKIDGVKLESTRVYQILAIYSTAASSLVLVVSLGEISFWMCSNGSLRCRICI

SEQ ID NO: 9 - protein, 558 aa, synthetic construct
  REGION 1..558: note = synthetically-generated protein
MAIIYLILLFTAVRGDQICIGYHANNSTEKVDTILERNVTVTHAKDILEKTHNGKLCKLNGIPPLELGDCSIAGWLLGNPECDRLLVPEWSYIMEKENPRGLCYPGSFNDYEELKHLLSSVKHFEKVKILPKDRWTQHTTTGGSRACAVSGNPSFFRNMVWLTKKGSNYPVAKGSYNNTSGEQMLIIWGVHHPNDETEQRTLYQNVGTYVSVTSTLNKRSTPEIARPKVNGLGSRMEFSWTLLDMWDTINFESTGNLIAPEYGFKISKRGSSGIMKTEGTLENCETKCQTPLGAINTTLPFHNVHPLTIGECPKYVKSEKLVLATGLRNVPQIESRGLFGAIAGFIEGGWQGMVDGWYGYHHSNDQGSGYAADKESTQKAFDGITNKVNSVIEKMNTQFEAVGKEFSNLERRLENLNKKMEDGFLDVWTYNAELLVLMENERTLDFHDSNVKNLYDKVRMQLRDNVKELGNGCFEFYHKCDDECMNSVKNGTYDYPKYEEESKLNRNEIKGVKLSSMGVYQILAIYATVAGSLSLAIMMAGISFWMCSNGSLQCRICI

SEQ ID NO: 10 - protein, 562 aa, synthetic construct
  REGION 1..562: note = synthetically-generated protein
MVIIYLILLFTAVRGDKICIGYHANNSTEMVDTILERNVTVTHAKDILEKTHNGKLCKLNGIPPLELGNCSIAGWLLGNPECDRLLRVPEWSYIMEKENPRDGLCYPGSFNDYEELKHFLSSVKHFEKVKILPKDRWTQHTTTGGSRACAVSGNPSFFRNMVWLTKKGSNYPVAQGSYNNTSGEKMLIIWGVHHPNDETEQRTLYQNVGTYVSVGTSTLNKRSTPDIATRPKVNGLGGRMEFSWTLLDMWDTINFESTGNLIAPEYGFKISKRGRSGIMKTEGTLENCETKCQTPLGAINTTLPFHNVHPLAIGECPKYVRSEKLVLATGLRNVPQIESRGLFGAIAGFIEGGWQGMIDGWYGYHHSNDQGSGYAADKESTQRAFDGITNKVNSVIEKMNTQFESVGKEFSNLERRLENLNKKMEDGFLDVWTYNAELLVLMENERTLGFHDSNVKNLYNKVRMQLRDNVKELGDGCFEFYHKCNDECMNSVKNGTYYYPKYEEESKLNRNEIKGVKLSSMGIYQILAIYATVAGSLSLAIMMAGISFWMCSNGSLQFRICI

SEQ ID NO: 11 - protein, 562 aa, synthetic construct
  REGION 1..562: note = synthetically-generated protein
MAIIYLILLFATVRGDQICIGYHANNSTETVDTILERNVTVTHAKDILEKAHNGKLCKLNGIPPLELGDCSIAGWLLGNPKCDRLLSVPEWSYIMEKENPKYSLCYPGSLNDYEELKHLLSSVKHFEKVRILPKDGWTQHTTTGGSKACAVSGKPSFFRNMVWLTEKGSNYPVAKGSYNNTSGEQMLIIWGVHHPIDEAEQRALYQEVGTYVSASTSTLNKRSIPEIAARPKVNGLGSRMEFFWTLLDVWDTINFESTGNLVVPEYGFKISKRGSSGIMKTEGTLGNCETKCQTPLGAINTTLPFHNVHPLTIGECPRYVKSEKLVLATGLRNIPQIESRGLFGAIAGFIEGGWQGMVDGWYGYHHSNEQGSGYAADKESTQKAFDGITNKENSVIEKMNTQFEAVGKEFNNLEKRLENLNKRMEDGFLDVWTYNAELLVLMENERTLDFHDSNVKNLYEKVRMQLRDNVKELGNGCFEFYHKCDNECMDSVKNGTYDYPKYEEESKAKRNEIKGVKLSSMGVYQILAIYATVAGSLSLAIMVAGISFWMCSNGSLQCRICI

SEQ ID NO: 12 - protein, 562 aa, synthetic construct
  REGION 1..562: note = synthetically-generated protein
MAIIYFILLFTAVRGDQICIGYHANNSTEKVDTILERNVTVTHAKNILEKTHNGRLCKLNGIPPLELGDCSITGWLLGNPECDRLLSVPEWSYIMEKENPRYSLCYPGSFNDYEELKHLLSSVKHLEKVKILPKDGWTQHETDGGSKACAVSGEPSFFRNMVWLTKKGPNYPVAKRSYNNTSGEQMLIIWGVHHPNDEAEQRALYQKVGTYVSASTSTLNKRSTPEIAARPEVNGLGSRMEFSWTLLDVWDTISFESTGNLVAPEYGFKISKRGSSGIIKTEGTLGNCETKCQTPLGAINTTLPFHNVHPLTIGECPKYVKSEKLVLATGPRNVPQIESRGLFGAIAGFIEGGWQGMVDGWYGYHHSKEQGSGYAADKESTQKAFDRITNKVNSVIEKINTQFEAVGKEFSNLEKRLENLNKKMEDGFIDVWTYNAELLVLMENERILDFHDSNVKNLYDKVRMQLRDNAKELGNGCFEFYHKCDDECMNSVKNGTYDYPKYEEESKLKRNEIKGVELSSMGVYQILVIYATVAGSLSLAIMIAGISFWMCSNGSLQCRVCI

SEQ ID NO: 13 - protein, 562 aa, synthetic construct
  REGION 1..562: note = synthetically-generated protein
MAIIYLILLFTAVRGDQICIGYHANNSTEKVDTILERNVTVTHAKDILEKTHNGKLCKLNGIPPLELGDCSIAGWLLGNPECDRLLSVPEWSYIMEKENPRDGLCYPGSFNDYEELKHLLSSVKHFEKVKILPKDRWTQHTTTGGSRACAVSGNPSFFRNMVWLTKKGSNYPVAKGSYNNTSGEQMLIIWGVHHPNDETEQRTLYQNVGTYVSVGTSTLNKRSTPEIATRPKVNGLGSRMEFSWTLLDMWDTINFESTGNLIAPEYGFKISKRGSSGIMKTEGTLENCETKCQTPLGAINTTLPFHNVHPLTIGECPKYVKSEKLVLATGLRNVPQIESRGLFGAIAGFIEGGWQGMVDGWYGYHHSNDQGSGYAADKESTQKAFDGITNKVNSVIEKMNTQFEAVGKEFSNLERRLENLNKKMEDGFLDVWTYNAELLVLMENERTLDFHDSNVKNLYDKVRMQLRDNVKELGNGCFEFYHKCDDECMNSVKNGTYDYPKYEEESKLNRNEIKGVKLSSMGVYQILAIYATVAGSLSLAIMMAGISFWMCSNGSLQCRICI

SEQ ID NO: 14 - protein, 562 aa, synthetic construct
  REGION 1..562: note = synthetically-generated protein
MAIIYLILLFATVRGDQICIGYHANNSTETVDTILERNVTVTHAKNILEKTHNGKLCKLNGIPPLELGDCSIAGWLLGNPECDRLLRVPEWSYIMEKENPRYSLCYPGSLNDYEELKHLLSSVKHFEKVRILPKDGWTQHTTTGGSKACAVSGKPSFFRNMVWLTKKGPNYPVAKRSYNNTSGEQMLIIWGVHHPNDEAEQRALYQKVGTYVSASTSTLNKRSTPDIATRPKVNGQGGRMEFSWTLLDVWDTINFESTGNLVAPEYGFKISKRGSSGIMKTEGTLGNCETKCQTPLGAINTTLPFHNVHPLTIGECPKYVKSEKLVLATGPRNVPQIESRGLFGAIAGFIEGGWQGMVDGWYGYHHSNDQGSGYAADKESTQKAFDRITNKVNSVIEKMNTQFEAVGKEFNNLEKRLENLNKKMEDGFLDVWTYNAELLVLMENERTLDFHDSNVKNLYEKVRMQLRDNVKELGNGCFEFYHKCDNECMDSVKNGTYDYPKYEEESKLKRNEIKGVKLSSMGIYQILAIYATVAGSLSLAIMIAGISFWMCSNGSLQCRICI

SEQ ID NO: 15 - protein, 562 aa, synthetic construct
  REGION 1..562: note = synthetically-generated protein
MAIIYFILLFTAVRGDQICIGYHANNSTEKVDTILERNVTVTHAKNILEKTHNGKLCKLNGIPPLELGDCSIAGWLLGNPECDRLLSVPEWSYIMEKENPKYSLCYPGSFNDYEELKHLLSSVKHFEKVKILPKDGWTQHETDGGSKACAVSGEPSFFRNMVWLTEKGSNYPVAKGSYNNTSGEQMLIIWGVHHPIDEAEQRALYQEVGTYVSASTSTLNKRSIPEIAARPKVNGLGGRMEFSWTLLDVWDTISFESTGNLVAPEYGFKISKRGSSGIMKTEGTLENCETKCQTPLGAINTTLPFHNVHPLTIGECPKYVKSEKLVLATGPRNVPQIESRGLFGAIAGFIEGGWQGMVDGWYGYHHSNDQGSGYAADKESTQRAFDGITNKVNSVIEKMNTQFEAVGKEFSNLEKRLENLNKKMEDGFLDVWTYNAELLVLMENERTLDFHDSNVKNLYNKVRMQLRDNVKELGNGCFEFYHKCDDECMSSVKNGTYDYPKYEEESKLKRNEIKGVKLSSMGVYQILAIYATVAGSLSLAIMVAGISFWMCSNGSLQCRICI

SEQ ID NO: 16 - protein, 564 aa, synthetic construct
  REGION 1..564: note = synthetically-generated protein
MKTIIALSYILCLVFAQKLPGNDNNSTATLCLGHHAVPNGTIVKTITNDQIEVTNATELVQSSTGEICDSPHQILDGENCTLIDALLGDPQCDGFQNKKWDLFVERSKAYSNCYPYDVPDYASLRSLVASSGTLEFNNESFNWTGVTQNGTSSACIRRSNSFFSRLNWLTHLNFKYPALNVTMPNNEQFDKLYIWGVHHPGTDKDQIFLYAQSGRITVSTKRSQQAVIPNIGSRPRRIPSRISIYWTIVKPGDILLINSTGNLIAPRGYFKIRSGKSSIMRSDAPIGKCSECITPNGSIPNDKPFQNVNRITYGACPRYVKQTLKLATGMRNVPEKQTRGIFGAIAGFIENGWEGMVDGWYGFRHQNSEGRGQAADLKSTQAAIDQINGKLNRLIGKTNEKFHQIEKEFSEVEGRIQDLEKYVEDTKIDLWSYNAELLVALENQHTIDLTDSEMNKLFEKTKKQLRENAEDMGNGCFKIYHKCDNACIGSIRNGTYDHDVYRDEALNNRFQIKGVELKSGYKDWILWISFAISCFLLCVALLGFIMWACQKGNIRCNIRCNICI

SEQ ID NO: 17 - protein, 566 aa, synthetic construct
  REGION 1..566: note = synthetically-generated protein
MKTIIALSHILCLVFAQKIPGNDNSTATLCIGHHAVPNGMIVKTITNDRIEVTNATELVQNSSIGEICDSPHQILDGENCTLIDALLGDPHCDGFQNEKWDLFVERSKAFSNCYPYDVPDYASLRSLVASSGTLEFKNESFNWTGVAQNGTSSACIRRSSSSFFSRLNWLTHLNYTYPALNVTMPNKEQFDKLYIWGVHHPGTDKDQIFLYAQSSGRITVSTKRSQQTAIPNIGSRPRIRDIPSRISIYWTIVKPGDVLVINSNGNLIAPRGYFKIQSGKSSIMRSDAPIGKCKSECITPNGSISNDKPFQNVNKITYGACPRYVKHSTLKLATGMRNVPEKQTRGLFGAIAGFIENGWEGMKDGWYGFRHQNSEGRGQAADLKSTQAAINQINGKLNRLIGKTNEKFHQIEKEFSEVEGRVQDLEKYVEDSKIDLWSYNAGLLVALENQHTIDLTDSEMNKLFERTRKQLRENAEDMGNGCFTIYHKCDNACIGSIRNGTYDHNVYRDEALNKRFQIKGIELKSGYKDWILWISFAISCFLLCVALLGFIMWACQKGNIRCNICI

SEQ ID NO: 18 - protein, 566 aa, synthetic construct
  REGION 1..566: note = synthetically-generated protein
MKTIIALSYIFCLVFAQKLPGNDNSTAMLCLGHHAVPNGTLVKTITNDQIEVTNATELVQSSSTGRICDSPHRILDGKNCTLMDALLGDPHCDGFQNKEWDLFVERSKAYSNCYPYDVPDYVSLRSLVASSGTLEFNNESFNWAGVTQNGTSSACKRRSNSSFFSRLNWLTHLNFKYPALNVTMPNNEQFDKLYIWGVHHPSTDSDQISLYAQASGRVTVSTKRSQQAVIPNIGSRPRIRNIPSRISIYWTIVKPGDILVINSNGNLIAPRGYFKIRNGKSSIMRSNAPIGKCNSECITPNGSIPNDKPFQNVNRVTYGACPRYVKQSTLKLATGMRNVPEKQTRGIFGAIAVFIENGWEGMVDGWYGFRHQNSEGTGQAADLKSTQAAVDQINGKLNRLIEKTNEKFHQIEKEFTEVEGRIQDLEKYVEDTKVDLWSYNAELLVALENQHTIDLTDAEMNKLFERTKKQLRENAEDIGNGCFKIYHKCDNACIESIRNGTYDHDVYRDEALNNRFHIKGVELKSGYKNWILWISFAISCFLLCVVLLGFIMWACQKGNIRCSICI

SEQ ID NO: 19 - protein, 566 aa, synthetic construct
  REGION 1..566: note = synthetically-generated protein
MKTIIALSYILCLVFAQKLPENDNSTATLCLGHHAVPNGTIVKTITNDQTEVTNATELVQSSSTGEICNSPHQILDGKNCTLIDALLGDPQCDGFQNKKWDLFVERSKAHSNCYPYDVPDYASLRSLIASSGTLEFNNESFNWTGVTQNGTSSACIRRSNNSFFSRLNWLTHLKFKYPALNVTMPNNEKFDKLYIWGVHHPGTDNDQIFLYAQASGRITVSTKRSQQTVIPNIGSRPRVRNIPSRVSIYWTIVKPGDILLINSTGNLIAPRGYFKIRSGKSSIMRSDAPIGKCNSACITPNGSIPNGKPFQNVNRITYGACPRYVKQNTLKLATGMRNVPERQTRGIFGAIAGFIENGWEGMMDGWYGFRHQNSEGIGQAADLKSTQAAIDQINGKLNRVIEKTNEKFHQIEKEFSEVEGRIQDIEKYVEDTKIDLWSYNAEFLVALENQHTIHLTDSEMNKLFEKTKKQLRENAEDMGNGCFKIYHKCNNACIGSIRNETYDHNVYRDEALNNRFQIKGVELKSGYKDWVLWISFAISCFLLCIVLLGFIMWACQRGNIRCNICI

SEQ ID NO: 20 - protein, 566 aa, synthetic construct
  REGION 1..566: note = synthetically-generated protein
MKTIIALSYILCLVFAQKLPGNDNSTATLCLGHHAVPNGTIVKTITNDQIEVTNATELVQNSSIGEICDSPHQILDGENCTLIDALLGDPQCDGFQNKKWDLFVERSKAYSNCYPYDVPDYASLRSLVASSGTLEFNNESFNWTGVTQNGTSSACIRRSNNSFFSRLNWLTHLNFKYPALNVTMPNNEQFDKLYIWGVHHPGTDKDQIFLYAQSSGRITVSTKRSQQAVIPNIGSRPRIRDIPSRISIYWTIVKPGDILLINSTGNLIAPRGYFKIRSGKSSIMRSDAPIGKCKSECITPNGSIPNDKPFQNVNRITYGACPRYVKQNTLKLATGMRNVPEKQTRGIFGAIAGFIENGWEGMVDGWYGFRHQNSEGRGQAADLKSTQAAIDQINGKLNRLIGKTNEKFHQIEKEFSEVEGRIQDLEKYVEDTKIDLWSYNAELLVALENQHTIDLTDSEMNKLFEKTKKQLRENAEDMGNGCFKIYHKCDNACIGSIRNGTYDHDVYRDEALNNRFQIKGVELKSGYKDWILWISFAISCFLLCVALLGFIMWACQKGNIRCNICI

SEQ ID NO: 21 - protein, 566 aa, synthetic construct
  REGION 1..566: note = synthetically-generated protein
MKTIIALSHILCLVFAQKIPGNDNSTAMLCLGHHAVSNGTIVKTITNDRIEVTNATELVQSSSTGEICDSPHRILDGKNCTLIDALLGDPHCDGFQNKEWDLFVERSKAHSNCYPYDVPDYVSLRSLVASSGTLEFKNESFNWTGVAQNGTSSACIRRSSSSFFSRLNWLTHLNYTYPALNVTMPNNEKFDKLYIWGVHHPGTDNDQIFLYAQASGRITVSTKRSQQTVIPNIGSRPRVRNIPSRISIYWTIVKPGDVLVINSNGNLIAPRGYFKIQSGKSSIMRSDAPIGKCNSECITPNGSISNDKPFQNVNKITYGACPRYVKHSTLKLATGMRNVPERQTRGIFGAIAVFIENGWEGMMDGWYGFRHQNSEGTGQAADLKSTQAAINQINGKLNRLIEKTNEKFHQIEKEFSEVEGRVQDLEKYVEDSKIDLWSYNAGLLVALENQHTIHLTDSEMNKLFERTKKQLRENAEDMGNGCFTIYHKCDNACIESIRNGTYDHNVYRDEALNKRFQIKGIELKSGYKDWVLWISFAISCFLLCVVLLGFIMWACQRGNIRCNICI

SEQ ID NO: 22 - protein, 566 aa, synthetic construct
  REGION 1..566: note = synthetically-generated protein
MRTIIALSYIFCLVFAQKLPENDNSTATLCIGHHAVPNGTLVKTITNDQVEVTNATELVQSSSTGGICDSPHQILDGKNCTLVDALLGDPHCDGFQNEKWDLFVERSKAFSNCYPYDVQDYASLRSLIASSGTLEFNNESFNWAGVTQNGTSSACKRRSNSSFFSRLNWLTHLKFKYPALNVTMPNKEQFDKLYIWGVHHPSTDSDQISLYAQASGRVTVSTKRSQQTAIPNIGSRPRIRNIPSRVSIYWTIVKPGDILLINCTGNLIAPRGYFKIRNGKSSIMRSNAPIGKCNSACITPNGSIPNGKPFQNVNRVTYGACPRYVKQSTLKLATGMRNVPEKQTRGLFGAIAGFIENGWEGMKDGWYGFRHQNSEGIGQAADLKSTQAAVDQINGKLNRVIEKTNEKFHQIEKEFTEVEGRIQDIEKYVEDTKVDLWSYNAELLVSLENQHTIDMTDSEMNKLFERTRKQLRENAEDIGNGCFKIYHKCNNACIGSIRNETYDHNVYRDEALNNRFHIKGVELKSGYKNWILWISFATSCFLLCIVLLGFIMWACQKGNIKCNICI

SEQ ID NO: 23 - protein, 573 aa, synthetic construct
  REGION 1..573: note = synthetically-generated protein
MEKIVLLLAIVSLVKSDQICIGYHANNSTEQVDTIMEKNVTVTHAQDILEKTHNGKLCDLDGVKPLILRDCSVAGWLLGNPMCDEFINVPEWSYIVEKANPANDLCYPGNFNDYEELKHLLSRINHFEKIQIIPKSSWSDHEASSGVSSACPYQGSSFFRNVVWLIKKNNTYPTIKRSYNNTNQEDLLVLWGIHHPNDAAEQTLYQNPTTYISVGTSTLNQRLVPKIATRSKVNGQSGRMEFFWTILKPNDAINFESNGNFIAPEYAYKIVKKGDSTIMKSELEYGNCNTKCQTPIGAINSSMPFHNIHPLTIGECPKYVKSNRLVLATGLRNSPQRERRRKKRGLFGAIAGFIEGGWQGMVDGWYGYHHSNEQGSGYAADKESTQKAIDGVTNKVNSIIDKMNTQFEAVGREFNNLERRIENLNKKMEDGFLDVWTYNAELLVLMENERTLDFHDSNVKNLYDKVRLQLRDNAKELGNGCFEFYHKCDNECMESVRNGTYDYPQYSEEARLKREEISGVKLESIGTYQILSIYSTVASSLALAIMVAGLSLWMCSNGSLQCRICIKFCEFRL

SEQ ID NO: 24 - protein, 566 aa, synthetic construct
  REGION 1..566: note = synthetically-generated protein
MEKIVLLLAIVSIVKSDQICIGYHANNSSEQVDTIMERNVTVTHAQDILEKTHNGKLCNLDGVKPLILRDCSVAGWLLGNPMCDEFLNVPEWSYIVEKINPANDLCYPGNFNDYEELKHLLSRITHFEKIQIIPKNSWSDHEASGVSSACPYQGRSSFFRNVVWLTKKDNAYPTIKRSYNNTNQEDLLVLWGIHHPNDAAEQTRLYQNPTTYISVGTSTLNQRLVPRIATRSKINGQSGRIEFFWTILKSNDAINFESNGNFIAPENAYKIVKKGDSTIMKSELEYGNCNTKCQTPIGAINSSMPLHNIHPLTIGECPKYVKSNRLVLATGLRNSPQGERRRKKRGLFGAIACFIEGGWQGMVDGWYGSHHSNDQGSGYAADKESTQRAIDGVTNKVNSIINKMNTQFEAVGREFNNLERRIGNLNKKMEDGFLDVWTYNAELLVLMGNERTLDFHDSNVKNLYDKVRLQLKDNAKELGNGCFEFYHRCDNECMESVRNGTYDYPQYSEEARLRREEISGVKLESIGVYQILSIYSTAASSLALAIMVAGLFLWMCSNGSLHADCI

SEQ ID NO: 25 - protein, 568 aa, synthetic construct
  REGION 1..568: note = synthetically-generated protein
MEKIVLLFAIVSLVKSDQICIGYHANNSTKQVDTIMEKNVTVTHAQDILEKKHNGKLCDLDGVRPLILRDCSVAGWLLGNPMCDEFINVPEWSYIVEKANPVNDLCYPGDFNDYEELKHLLSRINHFEKIQIIPKSSWSSHEASLGVSSACPYQGKSSFFRNVVWLIKKNNTYPTIKRSYNNTNQEDLLVMWGIHHPNDEAEQIKLYQNPTTYVSVGTSTLNQRLTPRIATRSKVNGQSGRMEFFWTILKPNDAINFESNGNFVAPEYAYKIVKKGDSAIMKSELEYSNCNTKCQTPMGAINSSMPFHHIHPLTIGECPKYVKSTRLVLATGLRNSPQRESRRKKRGLFGAIAGFIEAGWQGMVDGWYGYHHSNEQGSGYAADKESTQKAIDGVTNKVNSIIDKMNTQFEAIGREFNNLERRIENLNKKMEDGFLDVWTYKAELLVLMENERTLDYHDSNVRNLYDKVRLQLRDNTKELGNGCFEFYHKCDDECMESVKNGTYDYPQYSEEARLNREEISGVKLESIGIYQILSIYSTVASSLVLAIMVAGLSLWMCSNGSLQCRVCI

SEQ ID NO: 26 - protein, 574 aa, synthetic construct
  REGION 1..574: note = synthetically-generated protein
MEQIVLLLAIVSLVKSDHICIGYHANNSTEQVDTIMEKNVTVTHAQNILEKTHNGKLCDLDGVKPLILKDCSVAGWLLGNPMCDEFIRVPEWSYIVEKANPANDLCYPGSFNDYEELKHLLSRINHFEKLQIIPKSSWSDHEASSGVSSACPYQGTPSFFRNVVWLIKKNSTYPTIKKSYNNTNQEDLLILWGIHHSNDAAEQTKLYQNPTTYISIGTSTLNQRLVPKIATRSKVNGQSGRMDFFWTILKPNDAIHFESNGNFIAPEYAYKIVKEGDSAIMKSEVEYGNCNTKCQTPVGAINSSMPFHNIHPLTIGECPKYVKSNKLVLATGLRNSPLRERRRKRGLFGAIAGFIEGGWQGMVDGWYGFHHSNEQGSGYAADRESTQKAIDGVTNKVNSIIDKMNTQFEVVGREFNNLESRIENLNKKMEDGFLDVWTYNAELLVLMENERTLDFHDSNVKNLYDRVRLQLRDNAKELGNGCFEFYHKCDNECMESIRNGTYNYPQYSEEARLKREEISGVKLESIGTYQILSIYSTVASSLALAIMIAGLSLWMCSNGSLQCRICIYFCEFRL

SEQ ID NO: 27 - protein, 569 aa, synthetic construct
  REGION 1..569: note = synthetically-generated protein
MEKIVLLLAIVSLVKSDQICIGYHANNSTEQVDTIMEKNVTVTHAQDILEKTHNGKLCDLDGVKPLILRDCSVAGWLLGNPMCDEFINVPEWSYIVEKANPANDLCYPGNFNDYEELKHLLSRINHFEKIQIIPKSSWSDHEASSGVSSACPYQGRSSFFRNVVWLIKKNNTYPTIKRSYNNTNQEDLLVLWGIHHPNDAAEQTRLYQNPTTYISVGTSTLNQRLVPKIATRSKVNGQSGRMEFFWTILKPNDAINFESNGNFIAPEYAYKIVKKGDSTIMKSELEYGNCNTKCQTPIGAINSSMPFHNIHPLTIGECPKYVKSNRLVLATGLRNSPQGERRRKKRGLFGAIAGFIEGGWQGMVDGWYGYHHSNEQGSGYAADKESTQKAIDGVTNKVNSIIDKMNTQFEAVGREFNNLERRIENLNKKMEDGFLDVWTYNAELLVLMENERTLDFHDSNVKNLYDKVRLQLRDNAKELGNGCFEFYHKCDNECMESVRNGTYDYPQYSEEARLKREEISGVKLESIGTYQILSIYSTVASSLALAIMVAGLSLWMCSNGSLQCRICIK

SEQ ID NO: 28 - protein, 566 aa, synthetic construct
  REGION 1..566: note = synthetically-generated protein
MEKIVLLFAIVSLVKSDQICIGYHANNSTKQVDTIMEKNVTVTHAQDILEKTHNGKLCNLDGVKPLILKDCSVAGWLLGNPMCDEFLNVPEWSYIVEKINPANDLCYPGDFNDYEELKHLLSRINHFEKIQIIPKNSWSDHEASGVSSACPYQGTPSFFRNVVWLIKKNSTYPTIKKSYNNTNQEDLLILWGIHHSNDAAEQTKLYQNPTTYISIGTSTLNQRLTPRIATRSKVNGQSGRMDFFWTILKSNDAINFESNGNFIAPENAYKIVKKGDSAIMKSEVEYGNCNTKCQTPMGAINSSMPFHNIHPLTIGECPKYVKSNKLVLATGLRNSPLRERRRKRGLFGAIAGFIEGGWQGMVDGWYGFHHSNEQGSGYAADKESTQRAIDGVTNKVNSIINKMNTQFEAVGREFNNLERRIENLNKKMEDGFLDVWTYNAELLVLMENERTLDFHDSNVKNLYDKVRLQLKDNAKELGNGCFEFYHRCDNECMESIRNGTYNYPQYSEEARLNREEISGVKLESIGIYQILSIYSTAASSLALAIMVAGLFLWMCSNGSLQCRVCI

SEQ ID NO: 29 - protein, 568 aa, synthetic construct
  REGION 1..568: note = synthetically-generated protein
MEKIVLLLAIVSIVKSDQICIGYHANNSTKQVDTIMEKNVTVTHAQDILEKKHNGKLCDLDGVRPLILRDCSVAGWLLGNPMCDEFIRVPEWSYIVEKANPVNDLCYPGVFNDYEELKHLLSRINHFEKLQIIPKSSWSSHEASLGVSSACPYQGKSSFFRNVVWLTKKDNAYPTIKRSYNNTNQEDLLVMWGIHHPNDAAEQTKLYQNPTTYVSVGTSTLNQRLVPRIATRSKVNGQNGRMEFFWTILKSNDVINFESNGNFIAPEYAYKIVKEGDSAIMKSELEYSNCNTKCQTPMGAINSSMPFHNIHPLTIGECPKYVKSTRLVLATGLRNSPQRESRRKKRGLFGAIAGFIEGGWQGMVDGWYGFHHSNEQGSGYAADRESTQKAIDGVTNKVNSIINKMNTQFEAVGREFNNLERRIENLNKKMEDGFLDVWTYNAELLVLMENERTLDFHDSNVKNLYDKVRLQLRDNAKELGNGCFEFYHKCDNECMESVKNGTYDYPQYSEEARLNREEISGVKLESIGVYQILSIYSTVASSLALAIMIAGLSLWMCSNGSLQCRICI

SEQ ID NO: 30 - protein, 472 aa, synthetic construct
  REGION 1..472: note = synthetically-generated protein
MNPNQKIITIGSVCMTIGMANLILQIGNIISIWSHSIQLGNQNQIETCTICNQSVITYENNTWVNQTYVNISNTNFAAGQSVVSVKLAGNSSLCPVSGWAIYSKDNSIRIGSKGDVFVIREPFISCSPLECRTFFLTQGALLNDKHSNGTIKDRSPYRTLMSCPIGEVPSPYNSRFESVAWSASACHDGINWLTIGISGPDNGAVAVLKYNGIITDTIKSWRNNILRTQESECACVNGSCFTIMTDGPSDGQASYKIFRIEKGKIVKSVEMNAPNYHYEECSCYPDSSEITCVCRDNWHGSNRPWVSFNQNLEYQIGYICSGVFGDNPRPNDKTGSCGPVSSNGANGVKGFSFKYGNGVWIGRTKSISSRKGFEMIWDPNGWTGTDNFSIKQDIVGINEWSGYSGSFVQHPELTGLDCIRPCFWVELIRGRPKENTTIWTSGSSISFCGVNSDTVGWSWPDGAELPFTIDKY

SEQ ID NO: 31 - protein, 470 aa, synthetic construct
  REGION 1..470: note = synthetically-generated protein
MNPNQKIITIGSISIAIGIISLMLQIGNIISIWASHSIQTGSQNHTGICNQRIITYENSTWVNHTYVSINNTNVVAGKDKTSVTLAGNSSLCSISGWAIYTKDNSIRIGSKGDVFVIREPFISCSHLECKTFFLTQGALLNDKHSNGTVKDRSPYRALMSCPLGEAPSPYNSRFESIAWSASACHDGINWLTIGISGPDDGAVAVLKYNGIITGTIKSWKKQILRTQESECVCVNGSCFTVMTDGPSNGQASYKIFRIEKGKIVKSVEMNAPNYHYEECSCYPDSSEITCVCRDNWHASNRPWVSFNQNLDYQIGYICSGVFGDNPRPEDGEGSCNPVTVDGANGVKGFSYKYDNGVWIGRTKSNRLRKGFEMIWDPNGWTNTDSDFSVKQDVVAITDWSGYSGSFVQYPELTGLDCMRPCFWVELVRGLPRENTTIWTSGSSISFCGVNSDTANWSWPDGAELPFTIDK

SEQ ID NO: 32 - protein, 469 aa, synthetic construct
  REGION 1..469: note = synthetically-generated protein
MNPTQKIITIGSVCMTIGMANLILQIGNIISIWISHSIQLGNQNQIETCNQSIITYENNTWVNQTYVNISNTNFAAGQSVVSVKLAGNSSLCPVSGWAIYSKDNSIRIGSRGDVFVIRESFISCSHLECRTFFLTQGALLNDRHSNGTVKDRSPHRTLMSCPVGEAPSPYNSKFESVAWSASACHDGMGWLTIGISGPDNGAVAVLKYNGIITETIKSWKKRILRTQESECVCMNGSCFTIMTDGPSNGAASYKIFKIEKGKVTKSIELNAPNFHYEECSCYPDTGTVMCVCRDNWHGANRPWVSFNQNLEYQIGYICSGIFGDNPRPNDKTGSCGPVSSNGANGVKGFSFKYGNGVWIGRTKSISSRNGFEMIWDPNGWTGTDNNFSIKQDIVGIKEWSGYSGSFIQHPELTGLNCIRPCFWVELIRGRPKENTIWTSGSSISFCGVDSDTANWSWPDGAELPFIIDK

SEQ ID NO: 33 - protein, 469 aa, synthetic construct
  REGION 1..469: note = synthetically-generated protein
MNPNKKIITIGSICMTIGMANLMLQIGNIISIWVSHSIQIGNQSQIETCNQSVITYENNTWVNHTYVNINNTNVVAGEDKTSVTLAGNSSLCPIRGWAIYSKDNSVRIGSKGDVFVMREPFISCSPLECRTFFLTQGTLLNDKHSNGTIKDRSPYRTLMSCPIGEVPSPYNSRFESVAWSASACHDGTSWLTIGISGPDSGAVAVLKYNGIITDTIKSWRNNILRTQESECACVNGSCFTIMTDGPSDGQASYKIFRIEKGKIIKSVEMKAPNYHYEECSCYPDTGIVMCVCRDNWHGSNRPWVSFNQNLEYQMGYICSGVFGDNPRPKDGKGSCNPVTVDGADGVKGFSYKYGNGVWIGRTKSISSRKGFEMIWDTNGWTGTDNKFSIKQDIVGINEWSGYSGSFVQHPELTGLDCIRPCFWVELIRGRPEENTIWTSGSIISFCGVNSDTVGWSWPDGAELPFTVDK

SEQ ID NO: 34 - protein, 469 aa, synthetic construct
  REGION 1..469: note = synthetically-generated protein
MNPNQKIITIGSVCMTIGMANLILQIGNIISIWISHSIQLGNQNQIETCNQSVITYENNTWVNQTYVNISNTNFAAGQSVVSVKLAGNSSLCPVSGWAIYSKDNSIRIGSKGDVFVIREPFISCSPLECRTFFLTQGALLNDKHSNGTIKDRSPYRTLMSCPIGEVPSPYNSRFESVAWSASACHDGINWLTIGISGPDNGAVAVLKYNGIITDTIKSWRNNILRTQESECACVNGSCFTIMTDGPSDGQASYKIFRIEKGKIVKSVEMNAPNYHYEECSCYPDSSEITCVCRDNWHGSNRPWVSFNQNLEYQIGYICSGIFGDNPRPNDKTGSCGPVSSNGANGVKGFSFKYGNGVWIGRTKSISSRKGFEMIWDPNGWTGTDNNFSIKQDIVGINEWSGYSGSFVQHPELTGLDCIRPCFWVELIRGRPKENTIWTSGSSISFCGVNSDTVGWSWPDGAELPFTIDK

SEQ ID NO: 35 - protein, 470 aa, synthetic construct
  REGION 1..470: note = synthetically-generated protein
MNPTQKIITIGSISIAIGIISLMLQIGNIISIWASHSIQTGSQNHTGICNQRIITYENSTWVNHTYVNINNTNVVAGKDKTSVTLAGNSSLCPIRGWAIYSKDNSVRIGSKGDVFVMREPFISCSHLECRTFFLTQGTLLNDKHSNGTVKDRSPYRALMSCPLGEAPSPYNSKFESVAWSASACHDGMGWLTIGISGPDSGAVAVLKYNGIITGTIKSWKKQILRTQESECVCVNGSCFTVMTDGPSNGAASYKIFKIEKGKVTKSIELNAPNFHYEECSCYPDTGTVMCVCRDNWHGANRPWVSFNQNLDYQIGYICSGVFGDNPRPEDGEGSCNPVTVDGANGVKGFSYKYGNGVWIGRTKSISSRNGFEMIWDPNGWTNTDSDFSVKQDVVAITDWSGYSGSFIQHPELTGLDCMRPCFWVELVRGLPRENTTIWTSGSSMSFCGVNSDTANWSWPDGAELPFIIDK

SEQ ID NO: 36 - protein, 469 aa, synthetic construct
  REGION 1..469: note = synthetically-generated protein
MNPNKKIITIGSICMTIGMANLMLQIGNIISIWVSHSIQIGNQSQIETCNQSIITYENNTWVNHTYVSINNTNVVAGEDKTSVTLAGNSSLCSISGWAIYTKDNSIRIGSRGDVFVIREPFISCSHLECKTFFLTQGALLNDRHSNGTVKDRSPHRTLMSCPVGEAPSPYNSRFESVAWSASACHDGTSWLTIGISGPDDGAVAVLKYNGIITETIKSWKKRILRTQESECVCMNGSCFTIMTDGPSNGQASYKIFRIEKGKIIKSVEMKAPNYHYEECSCYPDTGIVMCVCRDNWHGSNRPWISFNQNLEYQMGYICSGVFGDNPRPKDGKGSCNPVTVDGADGVKGFSYKYDNGVWIGRTKSNRLRKGFEMIWDSNGWTGTDNKFSIKQDIVGIKEWSGYSGSFIQHPELTGLNCIRPCFWVELIRGRPEENTIWTSGSSISFCGVDSDTANWSWPDGAELPFTVDK

SEQ ID NO: 37 - protein, 469 aa, synthetic construct
  REGION 1..469: note = synthetically-generated protein
MNPNQKIITIGSVSLTISTICFFMQIAILITTVTLHFKQYEFNSPPNNQVMLCEPTTIIERNITEIVYLTNTTIEKEICPKPAEYRNWSKPQCITGFAPFSKDNSIRLSAGGDIWVTREPYVSCDPDKCYQFALGQGTTLNNVHSNNTVRDRTPYRTLLMNELGVPFHLGTKQVCIAWSSSSCHDGKAWLHVCITGDDKNATASFIYNGRLVDSVVSWSKYILRTQESECVCINGTCTVVMTDGSASGKADTKILFIEEGKIVHTSTLSGSAQHVEECSCYPRYPGVRCVCRDNWKGSNRPIVDINIKDHSIVSSYVCSGLVGDTPRKNDSSSSSHCLDPNNEEGGHGVKGWAFDDGNDVWMGRTINETSRLGYETFKVIEGWSNPKSKLQINRQVIVDRGDRSGYSGIFSVEGKSCINRCFYVELIRGRKEETEVLWTSNSIVVFCGTSGTYGTGSWPDGADLNLMPI

SEQ ID NO: 38 - protein, 469 aa, synthetic construct
  REGION 1..469: note = synthetically-generated protein
MNPNQKIIAIGSVSLTIATICFLMQIAILVTTVTLHFKQYECNSPPNNQVMPCEPIIIERNITEIVYLNNTTIEKEICPKLAEYRNWSKPQCNITGFAPFSKDNSIRLSASGDIWVTREPYVSCDPDKCYQFALGQGTTLNNGHSNDTVHDRIPHRTLLMNELGVPFHLGTRQVCIAWSSSSCHDGKAWLHVCVTGHDENATASFIYDGRLVDSIGSWSKKILRTQESECVCINGTCTVVMTDGSASGRADTKILFIEEGKIVHISPLSGSAQHVEECSCYPRYSGVRCVCRDNWKGSNRPIVDINVKDYSIVSSYVCSGLVGDTPRKNDRSSSSYCRNPNNEKGSHGVKGWAFDNGDDVWMGRTISEKLRSGYETFKVIEGWSKPNSKLQINRQVIVERGNRSGYSGIFSVEGKNCINRCFYVELIRGREQETRVWWTSNSIIVFCGTSGTYGTGSWPDGADINLMPI

SEQ ID NO: 39 - protein, 469 aa, synthetic construct
  REGION 1..469: note = synthetically-generated protein
MNPNKKIITIGSVSLTISTICFFMQIAILITTVTLHFKQHECNSPPNNQVMLCEPTIIERNMTEIVYLTNITIEKEICPKPAEYRNWSKPQCGITGFAPFSRDNSIRLSAGGNIWVTREPYVSCDPNKCYQFALGQGTTLNNVHSNNTVRDRTPYRTLLMSELGVPFHLGTKQVCMAWSSSSCHDGKAWLHVCITGDDKNATASIIYNGRLVDSVVSWSKDILRTQESECVCIDGTCTVVMTDGNATGKADTKILFIKEGKIVHTSKLSGSAQHVEECSCYPRYPDVRCICRDNWKGSNRPIVDINIKDHSIVSSYVCSGLVGDTPRKSDSSSSSHCLNPNNEEGGHRVKGWAFDDGDDVWMGRTINETSRLGYETFKVVEGWSNPKSKLQINRQVIVDRGDRSGYSGIFSVESKSCINRCFYVELIRGRKQETEVWWTSNSIVVFCGTSGTYGTGSWPDGADLNLMHI

SEQ ID NO: 40 - protein, 469 aa, synthetic construct
  REGION 1..469: note = synthetically-generated protein
MNPNQKIITIGSVSLTIATVCFLMQIAILATTVTLHFKQYEFNSPPNNQVVLCEPTIIERNITEIVYLTNTTIEKEICPKLVEYRNWSKPQCDITGFAPFSKDNSIRLSAGGDIWVTREPYVSCDPGKCYQFALGQGTTLNNRHSNDTVHDRTPYRTLLMNELGIPFHLGTKQVCIAWSSSSCYDGKAWLHVCVTGDDKNATASFIYNGRLVDSIVSWSKEILRTQESECVCINGTCAVVMTDGSASGKADTKILFIEEGKIVHTSTLSGSAQHVEECSCYPRYPGVRCVCRDNWRGSNRPIVDINIKDYSIVSRYVCSGLVGDTPRKNDSSSSSHCLDPNNEEGGHGVKGWAFDDGNDVWMGRTISEKSRLGYETFKVIEGWSNPKSKLQTNRQVIVDRGNRSGYSGIFSVEGKSCINRCFFVELIRGRKEETEVLWTSNSIVVLCGTSGTYGAGSWPDGADLNLMPI

SEQ ID NO: 41 - protein, 469 aa, synthetic construct
  REGION 1..469: note = synthetically-generated protein
MNPNQKIITIGSVSLTISTICFFMQIAILITTVTLHFKQYEFNSPPNNQVMLCEPTIIERNITEIVYLTNTTIEKEICPKPAEYRNWSKPQCGITGFAPFSKDNSIRLSAGGDIWVTREPYVSCDPDKCYQFALGQGTTLNNVHSNNTVRDRTPYRTLLMNELGVPFHLGTKQVCIAWSSSSCHDGKAWLHVCITGDDKNATASFIYNGRLVDSVVSWSKEILRTQESECVCINGTCTVVMTDGSASGKADTKILFIEEGKIVHTSTLSGSAQHVEECSCYPRYPGVRCVCRDNWKGSNRPIVDINIKDHSIVSSYVCSGLVGDTPRKNDSSSSSHCLDPNNEEGGHGVKGWAFDDGNDVWMGRTINETSRLGYETFKVIEGWSNPKSKLQINRQVIVDRGDRSGYSGIFSVEGKSCINRCFYVELIRGRKEETEVLWTSNSIVVFCGTSGTYGTGSWPDGADLNLMPI

SEQ ID NO: 42 - protein, 469 aa, synthetic construct
  REGION 1..469: note = synthetically-generated protein
MNPNQKIISIGSVSLTIATICFLMQIAILVTTVTLHFKQYECNSPPNNQVMPCEPIIIERNITEIVYLNNTTIEKEICPKLAEYRNWSKPQCDITGFAPFSRDNSIRLSAGGNIWVTREPYVSCDPGKCYQFALGQGTTLNNGHSNDTVHDRTPYRTLLMSELGVPFHLGTRQVCIAWSSSSCYDGKAWLHVCVTGDDENATASFIYDGRLVDSVVSWSKDILRTQESECVCIDGTCTVVMTDGNATGKADTKILFIKEGKIVHTSKLSGSAQHVEECSCYPRYPDVRCICRDNWKGSNRPIVDINVKDYSIVSSYVCSGLVGDTPRKSDSSSSSHCLNPNNEEGGHGVKGWAFDNGDDVWMGRTISEKSRLGYETFKVVEGWSNPKSKLQTNRQVIVDRGNRSGYSGIFSVESKSCINRCFFVELIRGRKQETEVWWTSNSIVVLCGTSGTYGAGSWPDGADINLMPI

SEQ ID NO: 43 - protein, 469 aa, synthetic construct
  REGION 1..469: note = synthetically-generated protein
MNPNKKIITIGSVSLTIATVCFLMQIAILATTVTLHFKQHECNSPPNNQVVLCEPTIIERNMTEIVYLTNITIEKEICPKLVEYRNWSKPQCNITGFAPFSKDNSVRLSAGGDIWVAREPYVSCDPNKCYQFALGQGTTLNNRHSNDTVHDRIPHRTLLMNELGIPFHLGTKQVCMAWSSSSCHDGKAWLHVCVTGDDKNATASIIYNGRLVDSIGSWSKKILRTQESECVCINGTCAVVMTDGSASGRADTKILFIEEGKIVHISPLSGSAQHVEECSCYPRYPGVRCICRDNWKGSNRPIVDINIKDYSIVSRYVCSGLVGDTPRKNDRSSSSYCRNPNNEKGSHGVKGWAFDDGDDVWMGRTISEKLRSGYETFKVIEGWSKPNSKLQINRQVIVERGNRSGYSGIFSVEGKNCINRCFYVELIRGREQETRVWWTSNSIIVFCGTSGTYGTGPWPDGADLNLMHI

SEQ ID NO: 44 - protein, 584 aa, synthetic construct
  REGION 1..584: note = synthetically-generated protein
MKAIIVLLMVVTSNADRICTGITSSNSPHVVKTATQGEVNVTGVIPLTTTPTKSHFANLKGTETRGKLCPKCLNCTDLDVALGRPKCTGKIPSARVSILHEVRPVTSGCFPIMHDRTKIRQLPNLLRGYEHVRLSTHNVINAEAPGGPYKIGTSGSCPNITNGNGFFATMAWAVPKNDKNKTATNPLTIEVPYICTEGEDQITVWGFHSDNETQMAKLYGDSKPQKFTSSANGVTTHYVSQIGGFPNQTEDGGLPQSGRIVVDYMVQKSGKTGTITYQRGILLPQKVWCASGRSKVIKGSLPLIGEADCLHEKYGGLNKSKPYYTGEHAKAIGNCPIWVKTPLKLANGTKYRPPAKLLKERGFFGAIAGFLEGGWEGMIAGWHGYTSHGAHGVAVAADLKSTQEAINKITKNLNSLSELEVKNLQRLSGAMDELHNEILELDEKVDDLRADTISSQIELAVLLSNEGIINSEDEHLLALERKLKKMLGPSAVEIGNGCFETKHKCNQTCLDRIAAGTFDAGEFSLPTFDSLNITAASLNDDGLDNHTILLYYSTAASSLAVTLMIAIFVVYMVSRDNVSCSICL

SEQ ID NO: 45 - protein, 584 aa, synthetic construct
  REGION 1..584: note = synthetically-generated protein
MKAIIVLLMVVTSNADRICTGITSSNSPHVVKTATQGEVNVTGVIPLTTTPTKSHFANLKGTETRGKLCPKCLNCTDLDVALGRPKCTGKIPSARVSILHEVRPVTSGCFPIMHDRTKIRQLPNLLRGYEHIRLSTHNVINAEAPGGPYKIGTSGSCPNITNGNGFFATMAWAVPKNDKNKTATNPLTIEVPYICTEGEDQITVWGFHSDNETQMAKLYGDSKPQKFTSSANGVTTHYVSQIGGFPNQTEDGGLPQSGRIVVDYMVQKSGKTGTITYQRGILLPQKVWCASGRSKVIKGSLPLIGEADCLHEKYGGLNKSKPYYTGEHAKAIGNCPIWVKTPLKLANGTKYRPPAKLLKERGFFGAIAGFLEGGWEGMIAGWHGYTSHGAHGVAVAADLKSTQEAINKITKNLNSLSELEVKNLQRLSGAMDELHNEILELDEKVDDLRADTISSQIELAVLLSNEGIINSEDEHLLALERKLKKMLGPSAVEIGNGCFETKHKCNQTCLDRIAAGTFDAGEFSLPTFDSLNITAASLNDDGLDNHTILLYYSTAASSLAVTLMIAIFVVYMVSRDNVSCSICL

SEQ ID NO: 46 - protein, 585 aa, synthetic construct
  REGION 1..585: note = synthetically-generated protein
MKAIIVLLMVVTSSADRICTGITSSSSPHVVKTATQGEINVTGVIPLTTTPIKSHFANLKGTETRGKLCPKCPNCTDLDVALGRPKCTGKIPSARVSILHEARPVTSGCFPIMHDRTKIRQLPNLLRGYEHVRLSTHNVINAEDAPGGPYKIGTSGSCPNITNGNGFFATMAWAVPKNDKNKTATNPLTIEVPYVCTEGEDQITVWGFHSDNEAQMAKLYGDSKPQKFTSSANGVATHYVSQIGGFPNQTEDGGLPQSGRIIVDYMVQKPGKTGTIVYQRGILLPQKVWCTSGRSKVIKGFLPLIGEADCLHEKYGGLNKSRPYYTGEHAKAVGNCPIWVKTPLKLANGTKYRPPAKLLKEKGFFGAIAGFLEGGWEGMVAGWHGYTSHGAHGIAVAADLKSTQEAINRITKNLNSLSELEVKNLQRLSSAMDELHNEILELDEKVDDLRADTISSQIAEAVHFSNEGIINSEDEHLMALERKLKKMLGPSAVEIGNGCFETQHKCNQTCLDKIAAGTFDAEEFSLPTFDSLNITAASLDDDGLDNHTILLYYSTAASSLAVTLMIAIFIVYMISRDNVSCSICL

SEQ ID NO: 47 - protein, 583 aa, synthetic construct
  REGION 1..583: note = synthetically-generated protein
MKAMIVLLMVVTSNADRICTGITSSNSPHIVKTATQGEVNVTGVIPLTTTPTKSHFANLKGTKTRGKLCPKCLNCTDLDVALGRPKCTGNIPSARVSILHEVRPVTSGCFPIMHDRTKITQLPNLLRGYEHIRLSTHNVINAENAPGGPYKIGTSGSCPNVTNGNGFFATMAWAVPDKNKTATNSLTIEVPYICTEGEDQITIWGFHSDNETQMAKLYGDSNPQKFTSSANGITTHYVSQIGGFPDQTEDGGLPQSGRIVVDYMVQKSGKTGTITYQRGILLPQKVWCVSGRSKVIKGSLPLIGEADCLHEKYGGLNKSKPYYTGEHAKAIGNCPIWVKTPLTLANGTKYRPPAKLLRERGFFGAIAGFLEGGWEGMIAGWHGYTSHGAHGVAVAADLKSTQEAINKITQNLNSLSELEIKNLQRLSGAMDELHNEIIELDEKVDDLRADTISSQIELTVLLSNEGIINNEDEHLLALERKLKKMLGPSAIEIGNGCFETKHKCNQTCIDRIAAGTFDAGEFSLPTFDSLNITAASLNDDGLDNHTIMLYYSTAASSLAVTLMIAIFVVYMVSRDNFSCSICL

SEQ ID NO: 48 - protein, 584 aa, synthetic construct
  REGION 1..584: note = synthetically-generated protein
MKTIIVLLMVVTSKADRICTGITSSNSPHVVKTATQGEVNVTGAIPLTTTPTKSYFANLKGTRTRGKLCPDCLNCTDLDVALGRPMCVGTTPSAKASILHEVRPATSGCFPIMHDRTKIRQLANLLRGYENIRLSTQNVIDAEKAPGGPYRLGTSGSCPNATSKSGFFATMAWAVPKDNNKNATNPLTVEVPYICTEGEDQITVWGFHSDNKTQMKNLYGDSNPQRFTSSANGVTTHYVSQIGDFPDQTEDGGLPQSGRIVVDYMMQKPGKTGTIVYQRGVLLPQKVWCASGRSKVIKGSLPLIGEADCLHEEYGGLNKSKPYYTGKHAKAIGNCPIWVKAPLKLANGTKYRPPAKLLKERGFFGAIAGFLEGGWEGMITGWHGYTSHGAHGVAIAADLKSTQEAINKITKNLNSLSELEVKNLQRLSGAMNELHNEILELDEKVDDLRADTISSQIELAVLLSNEGIINSEDEHLLALERRLKKMLGPSAVDIGNGCFETKHKCNQTCLDRIAAGTFNAGEFSLPTFDSLNITAASLNEDGLDNHTILLYYSTVASSLAVTLMLAIFIVYMVSRDNVSCSVCL

SEQ ID NO: 49 - protein, 585 aa, synthetic construct
  REGION 1..585: note = synthetically-generated protein
MKAIIVLLMVVTSNADRICTGITSSNSPHVVKTATQGEVNVTGVIPLTTTPTKSHFANLKGTETRGKLCPKCLNCTDLDVALGRPKCTGKIPSARVSILHEVRPVTSGCFPIMHDRTKIRQLPNLLRGYEHVRLSTHNVINAEDAPGGPYKIGTSGSCPNITNGNGFFATMAWAVPKNDKNKTATNPLTIEVPYICTEGEDQITVWGFHSDNETQMAKLYGDSKPQKFTSSANGVTTHYVSQIGGFPNQTEDGGLPQSGRIVVDYMVQKSGKTGTITYQRGILLPQKVWCASGRSKVIKGSLPLIGEADCLHEKYGGLNKSKPYYTGEHAKAIGNCPIWVKTPLKLANGTKYRPPAKLLKERGFFGAIAGFLEGGWEGMIAGWHGYTSHGAHGVAVAADLKSTQEAINKITKNLNSLSELEVKNLQRLSGAMDELHNEILELDEKVDDLRADTISSQIELAVLLSNEGIINSEDEHLLALERKLKKMLGPSAVEIGNGCFETKHKCNQTCLDRIAAGTFDAGEFSLPTFDSLNITAASLNDDGLDNHTILLYYSTAASSLAVTLMIAIFVVYMVSRDNVSCSICL

SEQ ID NO: 50 - protein, 584 aa, synthetic construct
  REGION 1..584: note = synthetically-generated protein
MKTIIVLLMVVTSSADRICTGITSSNSPHIVKTATQGEVNVTGAIPLTTTPTKSYFANLKGTRTRGKLCPDCLNCTDLDVALGRPMCVGTTPSAKASILHEVRPVTSGCFPIMHDRTKIRQLANLLRGYENIRLSTQNVIDAEKAPGGPYRLGTSGSCPNATSKSGFFATMAWAVPKDNNKNATNPLTVEVPYVCTEGEDQITVWGFHSDNKTQMKNLYGDSNPQKFTSSANGITTHYVSQIGGFPDQTEDGGLPQSGRIVVDYMMQKPGKTGTIVYQRGVLLPQKVWCVSGRSKVIKGSLPLIGEADCLHEEYGGLNKSKPYYTGKHAKAIGNCPIWVKTPLKLANGTKYRPPAKLLRERGFFGAIAGFLEGGWEGMIAGWHGYTSHGAHGIAVAADLKSTQEAINKITQNLNSLSELEIKNLQRLSGAMNELHNEILELDEKVDDLRADTISSQIELAVLLSNEGIINSEDEHLMALERKLKKMLGPSAVDIGNGCFETKHKCNQTCIDRIAAGTFNAGEFSLPTFDSLNITAASLDDDGLDNHTILLYYSTAASSLAVTLMLAIFIVYMVSRDNVSCSICL

SEQ ID NO: 51 - protein, 584 aa, synthetic construct
  REGION 1..584: note = synthetically-generated protein
MKTAIIVLLMVVTSKADRICTGITSSSSPHVVKTATQGEINVTGVIPLTTTPIKSHFANLKGTKTRGKLCPKCPNCTDLDVALGRPKCTGNIPSARVSILHEARPVTSGCFPIMHDRTKIRQLPNLLRGYEHIRLSTHNVINAENAPGGPYKIGTSGSCPNVTNGNGFFATMAWAVPDKNKTATNSLTIEVPYICTEGEDQITIWGFHSDNEAQMAKLYGDSKPQKFTSSANGVATHYVSQIGDFPDQTEDGGLPQSGRIVVDYMVQKPGKTGTIVYQRGILLPQKVWCVSGRSKVIKGSLPLIGEADCLHEKYGGLNKSKPYYTGEYAKAIGNCPIWVKTPLKLANGTKYRPPAKLLKEKGFFGAIAGFLEGGWEGMIAGWHGYTSHGAHGVAVAADLKSTQEAINKITKNLNSLSELEVKNLQRLSSAMDELHNEIIELDEKVDDLRADTISSQIELAVLLSNEGIINSEDEHLMALERKLKKMLGPSAIEIGNGCFETKHKCNQTCLDKIAAGTFDAGEFSLPTFDSLNITAASLNEDGLDNHTILLYYSTAASSLAVTLMIAIFIVYMISRDNVSCSICL

SEQ ID NO: 52 - protein, 586 aa, synthetic construct
  REGION 1..586: note = synthetically-generated protein
MKTAIIVLLMVVTSNADRVCTGITSSNSPHVVKTATQGEINVTGVIPLTTTPTRSHFANLKGTKTRGKLCPTCLNCTDLDVALGRPMCVGITPSAKASILHEVKPVTSGCFPIMHDRTKIRQLPNLLRGYENVRLSTHNVINAEGAPGGPYKIGTSGSCPNATSKIGFFATMAWAVPKNDNNKTATNPLTVEVPYICTEGEDQITVWGFHSDNKTQMKSLYGDSNPQKFTSSANGMTTHYVSQIGSFPDQTEDGGLPQSGRIIVDYMVQKSRKTGTITYQRGILLPQKVWCVSGRSKVIKGSLPLIGEADCLHEKYGGLNKSKPYYTGEHAKAVGNCPIWVKTPLKLANGTKYRPPAKLLRERGFFGAIAGFLEGGWEGMIAGWHGYTSHGAHGVAVAADLKSTQEAINKITKNLNSLSELEVKNLQRISGAMDELHNEILELDEKVDDLRADTISSQIELAVLLSNEGIINSEDEHLMALERKLKKMLGPSAIEIGNGCFETKHKCNQTCIDRIAAGTFNAGEFSLPTFDSLNITAASLNDDGLDSHTILLYYSTAASSLAVTLMIAIFVVYMISRDNVSCSICL

SEQ ID NO: 53 - protein, 585 aa, synthetic construct
  REGION 1..585: note = synthetically-generated protein
MKAIIVLLMVVTSNADRICTGITSSNSPHVVKTATQGEVNVTGVIPLTTTPTKSYFANLKGTRTRGKLCPDCLNCTDLDVALGRPMCVGTTPSAKASILHEVRPVTSGCFPIMHDRTKIRQLPNLLRGYEKIRLSTQNVIDAEKAPGGPYRLGTSGSCPNATSKIGFFATMAWAVPKKDNYKNATNPQTVEVPYICTEGEDQITVWGFHSDNKTQMKSLYGDSNPQKFTSSANGVTTHYVSQIGDFPDQTEDGGLPQSGRIVVDYMVQKPGKTGTIVYQRGVLLPQKVWCASGRSKVIKGSLPLIGEADCLHEEYGGLNKSKPYYTGKHAKAIGNCPIWVKTPLKLANGTKYRPPAKLLKERGFFGAIAGFLEGGWEGMIAGWHGYTSHGAHGVAVAADLKSTQEAINKITKNLNSLSELEVKNLQRLSGAMDELHNEILELDEKVDDLRADTISSQIELAVLLSNEGIINSEDEHLLALERKLKKMLGPSAVDIGNGCFETKHKCNQTCLDRIAAGTFNAGEFSLPTFDSLNITAASLNDDGLDNHTILLYYSTAASSLAVTLMLAIFIVYMVSRDNVSCSICL

SEQ ID NO: 54 - protein, 584 aa, synthetic construct
  REGION 1..584: note = synthetically-generated protein
MKAILVLLMVVTSNADRICTGITSSNSPYVVKTATQGEVNVTGAIPLTTTPTKSHFANLKGTKTRGKLCPKCLNCTDLDVALGRPKCTGNIPSAEVSILHEVRPVTSGCFPIMHDRTKIRQLANLLRGYENIRLSTQNVIDAEKAPGGPYKLGTSGSCPNATSKSGFFATMAWAVPKDNNKNATNPLTVEVPYICAEGEDQITVWGFHSDNKTQMKNLYGDSNPQKFTSSANGVTTHYVSQIGGFPDQTEDGGLSQSGRIVVDYMMQKPGKTGTITYQRGILLPQKVWCASGRSKVIKGSLPLIGEADCLHEKYGGLNKSKPYYTGEHAKAIGNCPIWVKTPLKLANGTKYRPPARLLKERGFFGAIAGFLEGGWEGMVAGWHGYTSHGAHGVAVAADLKSTQEAVNKITKNLNSLSELEVKNLQRLSGAMDELHDEILELDEKVDDLRADTISSQIELAVVLSNEGIINSEDEHLLSLERKLKKMLGPSAVEIGNGCFETKHKCNQTCLDRIAAGTFDAGEFSLPTFDSLNITAASLNDDGLDNHTILLYYSTAASSLTVTLMLAIFIVYMVSRDNISCSICL

SEQ ID NO: 55 - protein, 584 aa, synthetic construct
  REGION 1..584: note = synthetically-generated protein
MKAIIVLLMVVTSDADRICTGITSSNSPHVVKTATQGEINVTGVIPLTTTPTKSYFANLKGIRTRGKLCPDCINCTDLDVALGRPMCMGTTPSAKASILHEVRPITSGCFPIMHDRTKIRQLPNLLRGYEKIRLSTQNVIDAEKAPRGPYRLGTSGSCPNATSKIGFFATMAWAVPKDNYKNATNPQTVEIPYICTEGEDQITVWGFHSDDKTQMKSLYGDSNPQKFTSSANGMTTHYVSQIGDFPDQTEDGRLPQSGRIVVDYMVQKPEKTGTIVYQRGVLLPQKVWCVSGRSKVIKGALPLIGEADCLHEEYGGLNKSKPYYTGKHAKAIGDCPIWVKTPLELANGTKYRAPAKLLKERGFFGAIAGFLEGGWKGMIAGWHGYISHGAHGVAVAADLKSTQEAINKITRNLNSLSELEVKNLQRLSGAMDELHSEILELDEKVDDLRADTVSSQIELAVLLSNEGIIKSEDEHLLALERKLKKMLGPSAIDIGNGCFETTHKCNQTCLDRIAAGTFNAREFSLPTFDSLNITAAYLNDDGLDNHAILLYYSTAASSLAVTLMLAIFIVYVVSRDNVSCSICL

SEQ ID NO: 56 - protein, 584 aa, synthetic construct
  REGION 1..584: note = synthetically-generated protein
MKVIIVLLMVVMSNADRICTGITSSSSPHVVKTATQGEVNVTGVIPLTITPTKSYFANLKGTRTRGKLCPDCLNCTDLDVALGRPMCVGTTPSAKASILHEVKPVTSGCFPIMHDRTKIRQLPNFLRGYEKIRLSTKNVIDAEKAPGGPYRLGTSRSCPNATSKVGFFATMAWAVPKNNYKNATNPQTVEVPYICTEGEDQITVWGFHSDNKTQMKSLYGDSNPQRFTSSANGVTTHYVSQIGSFPDQTEDGGLPQSGRIVVDYMVQKPGKTGTIVYQRGVLFPQKVWCASGKSKVIKGSLPLIGEADCLHEEYGGLTKSKPYYTGKHAKAIGNCPIWVKTSLKLANGTKYRPPAKLLKERGLFGAIAGFLEGGWEGMIAGWHGYTSHGAHGVAVAADLKSTQEAINKITKNLNFLSELEVKNLQRLSGAMDELHNEILELDEKVDDLRADTMSSQIELAVLLSNEGIINSEDEHLLALERQLKKMLGPSAVDIGNGCFETKHKCNQTCLDKIAAGTFNAGEFSLPTFDSLNITAASLNNDGLDNHTILLYYSTVASSLAVTLMIAIFVVYMVSRDNVSCSICL

SEQ ID NO: 57 - protein, 584 aa, synthetic construct
  REGION 1..584: note = synthetically-generated protein
MKAIIVLLMVVTSNADRICTGITSSNSPHVVKTATQGEVNVTGVIPLTTTPTKSYFANLKGTRTRGKLCPDCLNCTDLDVALGRPMCVGTTPSAKASILHEVRPVTSGCFPIMHDRTKIRQLPNLLRGYEKIRLSTQNVIDAEKAPGGPYRLGTSGSCPNATSKIGFFATMAWAVPKDNYKNATNPQTVEVPYICTEGEDQITVWGFHSDNKTQMKSLYGDSNPQKFTSSANGVTTHYVSQIGDFPDQTEDGGLPQSGRIVVDYMVQKPGKTGTIVYQRGVLLPQKVWCASGRSKVIKGSLPLIGEADCLHEEYGGLNKSKPYYTGKHAKAIGNCPIWVKTPLKLANGTKYRPPAKLLKERGFFGAIAGFLEGGWEGMIAGWHGYTSHGAHGVAVAADLKSTQEAINKITKNLNSLSELEVKNLQRLSGAMDELHNEILELDEKVDDLRADTISSQIELAVLLSNEGIINSEDEHLLALERKLKKMLGPSAVDIGNGCFETKHKCNQTCLDRIAAGTFNAGEFSLPTFDSLNITAASLNDDGLDNHTILLYYSTAASSLAVTLMLAIFIVYMVSRDNVSCSICL

SEQ ID NO: 58 - protein, 583 aa, synthetic construct
  REGION 1..583: note = synthetically-generated protein
MKVIIVLLMVVTSDADRICTGITSSNSPHVVKTATQGEVNVTGVIPLTITPTKSYFANLKGTKTRGKLCPDCFNCTDLDVALGRPMCMGTTPSAKASILHEVKPVTSGCFPIMHDRTKIRQLANLLRGYENIRLSTQNVIDAEKAPRGPYRLGTSRSCPNATSKSGFFATMAWAVPKDNNKNATNPLTVEVPYICAEGEDQITVWGFHSDDKTQMKNLYGDSNPQRFTSSANGVTTHYVSQIGGFPDQTEDGGLPQSGRIVVDYMMQKPGKTGTIVYQRGVLFPQKVWCASGKSKVIKGSLPLIGEADCLHEKYGGLNKSKPYYTGEHAKAIGNCPIWVKTPLKLANGTKYRPPAKLLKERGFFGAIAGFLEGGWEGMIAGWHGYTSHGAHGVAVAADLKSTQEAINKITKNLNSLSELEVKNLQRLSGAMDELHSEILELDEKVDDLRADTISSQIELAVLLSNEGIINSEDEHLLALERKLKKMLGPSAVEIGNGCFETKHKCNQTCLDKIAAGTFNAGEFSLPTFDSLNITAASLNNDGLDNHTILLYYSTAASSLTVTLMLAIFIVYVVSRDNVSCSIC

SEQ ID NO: 59 - protein, 583 aa, synthetic construct
  REGION 1..583: note = synthetically-generated protein
MKAIIVLLMVVMSNADRICTGITSSNSPHVVKTATQGEVNVTGVIPLTTTPTKSHFANLKGTKTRGKLCPDCINCTDLDVALGRPMCVGTIPSAKASILHEVRPVTSGCFPIMHDRTKIRQLPNLLRGYEKIRLSTKNVIDAEKAPRGPYRLGTSGSCPNATSKVGFFATMAWAVPKNNYKNATNPQTVEIPYICTEGEDQITVWGFHSDNKIQMKNLYGDSNPQKFTSSANGVTTHYVSQIGSFPDQTEDGGLPQSGRIVVDYMVQKPEKTGTIVYQRGILLPQKVWCVSGRSKVIKGALPLIGEADCLHEKYGGLNKSKPYYTGKHAKAIGNCPIWVKTPLKLANGTKYRPPAKLLKERGFFGAIAGFLEGGWEGMIAGWHGYTSHGAHGVAVAADLKSTQEAINKITKNLNSLSELEVKNLQRLSGAMDELHDEILELDEKVDDLRADTISSQIELAVLLSNEGIINSEDEHLLALERKLKKMLGPSAIDIGNGCFETKHKCNQTCLDRIAAGTFDAGEFSLPTFDSLNITAASLNEDGLDNHTILLYYSTVASSLAVTLMIAIFVVYMVSRDNVSCSIC

SEQ ID NO: 60 - protein, 584 aa, synthetic construct
  REGION 1..584: note = synthetically-generated protein
MKAIIVLLMVVASDADRICTGITSSNSPHVVKTATQGEVNVTGVIPLTITPTKSYFANLKGIRTRGKLCPDCFNCTDLDVALGRPMCVGATPSAKASILHEVRPVTSGCFPIMHDRTKIRQLPNLLRGYENIRLSTQNVIDAEKAPRGPYRLGTSGSCPNTTSKIGFFATMAWAVPKDKYKNATNPQTLEIPYICTEGEDQITVWGFHSDNKTQMKNLYGDSNPQKFTSSANGVTTHYVSQIGDFPNQTEDGGLPQSGRIVVDYMVQKPGRTGTIVYQRGILLPQKVWCANGRSKVIKGALPLIGEADCLHEKYGGLNKSKPYYTGKHAKAIGNCPIWVKTPLKLANGTKYRPPAKLLKERGFFGAIAGFLEGGWEGMIAGWHGYTSHGAHGVAVAADLKSTQEAINKITKNLNSLSELEVKNLQRLSGAMDELHSEILELDEKVDDLRADTISSQIELAVLLSNEGIINSEDEHLLALERKLKKMLGPSAIDIGNGCFETKHKCNQTCLDRIAAGTFSAGEFSLPTFDSLNITAASLNDDGLDNHAILLYYSTAASSLTVTLMLAIFIVYMVSKDNVSCSICL

SEQ ID NO: 61 - protein, 467 aa, synthetic construct
  REGION 1..467: note = synthetically-generated protein
MLPSTIQTLTLFLTSGGVLLSLYVSASLSYLLYSDILLKFSPTEITAPTMPLDCANASNVQAVNRSATKGVTLLLLPEPEWTYPRLSCPGSTFQKALLISPHRFGETKGNSAPLIIREPFVACGPNECKHFALTHYAAQPGGYYNGTRGDRNKLRHLISVKLGKIPTVENSIFHMAAWSGSACHDGKEWTYIGVDGPDNNALLKVKYGEAYTDTYHSYANNILRTQESACNCIGGNCYLMITDGSASGVSECRFLKIREGRIIKEIFPTGRVKHTEECTCGFASNKTIECACRDNRYTAKRPFVKLNVETDTAEIRLMCTDTYLDTPRPNDGSITGPCESDGDKGSGGIKGGFVHQRMKSKIGRWYSRTMSKTERMGMGLYVKYGGDPWADSDALAFSGVMVSMKEPGWYSFGFEIKDKKCDVPCIGIEMVHDGGKETWHSAATAIYCLMGSGQLLWDTVTGVDMAL

SEQ ID NO: 62 - protein, 466 aa, synthetic construct
  REGION 1..466: note = synthetically-generated protein
MLPSTIQTLTLVLTSGGVLLSLYVSALLSYLLYSDILLKFSRTEITAPIMPLDCANASNVQAVNRSATKGVTLLLPGPEWTYPRLSCQGSTFQKALLISPHRFGEAKGNSAPLIIREPFIACGPKECKHFALTHYAAQPGGYYNGTREDRNKLRHLISVNLGKIPTVENSIFHMAAWSGSACHDGREWTYIGVDGPDSNALLKIKYGEAYTDTYHSYAKNILRTQESACNCIGGDCYLMITDGPASGISECRFLKIRKGRIIKEIFPTGRVEHTEECTCGFASNKTIECACRDNSYTAKRPFVKLNVEIDTAEIRLMCTETYLDTPRPDDGSITGPCESNGDKGSGGIKGGFVHQRMESKIGRWYSRTMSKTERMGMGLYVKYDGDPWADSGALAFSGVMVSMKEPGWYSFGFEIRDKKCDVPCIGIEMVHDGGRETWHSAATTIYCLMGSGQLLWDTVTGVNMTL

SEQ ID NO: 63 - protein, 466 aa, synthetic construct
  REGION 1..466: note = synthetically-generated protein
MLSSTIQTLTLLLTSGGVLLSLYVSASLSYLLYSDILLKFSQTEITAPIMSLDCANASNVQAVNRSAAKGVTLLLPEPEWTYPRLSCPGSIFQKALLISPHRFGEIKGNSAPLIIREPFIACGPTECKHFALTHYAAQPGGYYSGTRGDRNKLRHLISVKLGKIPTVETSIFHMAAWSGSSCHDGKEWTYIGVDGPDNNALLKIKYGEAYTDTYHSYANKILRTQESACNCIGGNCYLMITDGPASGVSECRFLKIREGRIIKEIFPTGRIKHTEECTCGFASNETIECACRDNNYTAKRPFVKLNVETDTAEIRLMCTKTYLDTPRPNDGSTTGPCESDGDKGSGGIKGGFVHQRMASKIGRWYSRTMSKTKRMGMGLYVKYDGDPWTDSEALALSGVMVSMEEPGWYSFGFEIKDKKCDVPCIGIEMVHDGGKTTWHSAATAVYCLMGSGQLLWDTVTGVDMAL

SEQ ID NO: 64 - protein, 466 aa, synthetic construct
  REGION 1..466: note = synthetically-generated protein
MLPSTIQTLTLFLTSGGVLLSIYVSASLSYLIYSDILLKFSPTEITAPTMPLDCANASNVHAVNRSATKGVTFLLPEPEWTYPRLSCPGSTFQKALLISPHRFGETKGNSAPLIIREPFVACGPNECKHFALTHYATQPGGYYNGTRGDRNKLRHLISVELGKIPTVENSIFHMTAWSGSACHDGKEWTYVGVDGPDNNALLKVKYGEAYTDTYHSYANNILRTQESACNCIRGNCYLMITDGSASGVSECRFLKIQEGRIIKEIFPTGRVKHTEECTCGFANNKTIECACRDNRYTAKRPFVKLSVETDTAEIRLMCTDTYLDTPRPNDGSITGPCESDGNEGSGGIKGGFVHQRMKSKIGRWYSRTMSQTERMGMGLYVKYGGDPWADSDALAFSGVMISMKEPGWYSFGFEMKDKKCDVPCIGVEMVHDGGKETWHSAATAIYCLMGSGKLLWDTVTGVNMAL

SEQ ID NO: 65 - protein, 466 aa, synthetic construct
  REGION 1..466: note = synthetically-generated protein
MLPSTIQTLTLFLTSGGVLLSLYVSASLSYLLYSDILLKFSPTEITAPTMPLDCANASNVQAVNRSATKGVTLLLPEPEWTYPRLSCPGSTFQKALLISPHRFGETKGNSAPLIIREPFVACGPNECKHFALTHYAAQPGGYYNGTRGDRNKLRHLISVKLGKIPTVENSIFHMAAWSGSACHDGKEWTYIGVDGPDNNALLKVKYGEAYTDTYHSYANNILRTQESACNCIGGNCYLMITDGSASGVSECRFLKIREGRIIKEIFPTGRVKHTEECTCGFASNKTIECACRDNRYTAKRPFVKLNVETDTAEIRLMCTDTYLDTPRPNDGSITGPCESDGDKGSGGIKGGFVHQRMKSKIGRWYSRTMSKTERMGMGLYVKYGGDPWADSDALAFSGVMVSMKEPGWYSFGFEIKDKKCDVPCIGIEMVHDGGKETWHSAATAIYCLMGSGQLLWDTVTGVDMAL

SEQ ID NO: 66 - protein, 466 aa, synthetic construct
  REGION 1..466: note = synthetically-generated protein
MLSSTIQTLTLVLTSGGVLLSLYVSALLSYLLYSDILLKFSQTEITAPIMPLDCANAPNVQAVNRSAAKGVTLLLPGPEWTYPRLSCQGSTFQKALLISPHRFGEIKGNSAPLIIREPFIACGPKECKHFALTHYATQPGGYYNGTREDRNKLRHLISVNLGKIPTVENSIFHMTAWSGSACHDGREWTYIGVDGPDSNALLKIKYGEAYTDTYHSYAKNILRTQESACNCIGGDCYLMITDGPASGISECRFLKIQEGRIIKEIFPTGRIKHTEECTCGLASNETIECACRDNSYTAKRPFVKLNVEIDTAEIRLMCTETYLDTPRPDDGSITGPCESNGDKGSGGIKGGFVHQRMASKIGRWYSRTMSKTKRMGMGLYVKYDGDPWTDSEALALSGVMVSMEEPGWYSFGFEIRDKKCDVPCIGVEMVHDGGKTTWHSAATAVYCLMGSGQLLWDTVTGVNMTL

SEQ ID NO: 67 - protein, 466 aa, synthetic construct
  REGION 1..466: note = synthetically-generated protein
MLPSTIQMLTLFLTSGGVLLSIYVSASLSYLIYSDILLKFSRTEITAPIMSLDCANASNVHAVNRSATKGVTFLLPEPEWTYPRLSCSGSTFQKALLISPHRFGEAKGNSAPLIVREPFIACGPTECKHFALTHYAAQPGGYYSGTRGDRNKLRHLISVELGKIPTVETSIFHMAAWSGSSCHDGKEWTYVGVDGPDNNALLKIKYGEAYTDTYHSYANKILRTQESACNCIRGNCYLMITDGPASGVSECRFLKIREGLIIKEIFPTGRVEHTEECTCGFANNKTIECACRDNNYTAKRPFVKLSVETDTAEIRLMCTKTYLDTPRPNDGSTTGPCESDGEKGSGGIKGGFVHQRMESKIGRWYSRTMSQTERMGMGLYVKYDGDPWADSGALAFSGVMISMKEPGWYTFGFEIKDKKCDVPCIGIEMVHDGGRETWHSAATTIYCLMGSGKLLWDTVTGVNMAL

SEQ ID NO: 68 - protein, 466 aa, synthetic construct
  REGION 1..466: note = synthetically-generated protein
MLPSTIQTLTLFLTSGGVLLSLYVSASLSYLLYSDILLKFSRTEVTAPIMPLDCANASNVQAVNRSATKGVTPLLPEPEWTYPRLSCPGSTFQKALLISPHRFGETKGNSAPLIIREPFIACGPKECKHFALTHYAAQPGGYYNGTREDRNKLRHLISVKLGKIPTVENSIFHMAAWSGSACHDGREWTYIGVDGPDSNALLKIKYGEAYTDTYHSYAKNILRTQESACNCIGGDCYLMITDGPASGISECRFLKIREGRIIKEIFPTGRVKHTEECTCGFASNKTIECACRDNSYTAKRPFVKLNVETDTAEIRLMCTKTYLDTPRPNDGSITGPCESDGNEGSGGIKGGFVHQRMASKIGRWYSRTMSKTQRMGMGLYVKYDGDPWTDSEALALSGVMVSMEEPGWYSFGFEIKDKKCDVPCIGIEMVHDGGKTTWHSAATAIYCLMGSGQLLWDTVTGVNMTL

SEQ ID NO: 69 - protein, 466 aa, synthetic construct
  REGION 1..466: note = synthetically-generated protein
MPPSTIQTLTLFLTSGGVLLSIYVSASLSYLLYLDILLKFPSTEITAPTMPLDCANASNVQAVNHSATKGVTLLLPEPEWTYPRLSCPGSTFQRALLISPHRFGETKGNSAPLIMREPFIACGPNECKHFALTHYTAQPGGYYNGTREDRNNLRHLISVKLGKIPTVENSIFHMAAWSGSACHDGKEWTYIGVDGPDNNALLKVKYGEAYTDTYHSYANKILRTQESACNCIGGNCYLMITDGSASGVSECRFLKIREGRIMKEIFPTGRTQHTEECTCGFASNKTIECACRDNSYTAKRPFVKLNVETDTAEIRLMCTETYLDTPRPDDGSITGPCESDGDEGSGGIKGGFVHQRMESKIGRWYSRTMSKTERKGMGLYVKYNGDPWADSDALAFSGVMVSMKEPGWYSFGFEIKDKKCDVPCIGIEMVHDGGKETWHSAATAIYCLMGSGQLLWDTVTGVDMAL

SEQ ID NO: 70 - protein, 466 aa, synthetic construct
  REGION 1..466: note = synthetically-generated protein
MLPSTIQTLTLLLTSGGVLLSLYVSASLSYLLYSDILLKFSRTEVTAPIMPLDCANASNVQAVNRSVTKGVTPLLPEPEWMYPRLSCPGSTFQKALLISPHRFGEIKGNSAPLIIREPFIACGPKECKHFALTHYATQPGGYYNGTREDRNKLRHLVSVKLGKIPTVENSMFHMAAWSGSACHDGREWTYIGVDGPDNNALLKIKYGETYTDTYHSYAKNILRTQESACNCIGGDCYLMITDGPASGVSECRFLKIREGRIVKEIFPTGRVKHTEECTCGFANNKTIECACRDNRYTAKRPFVKLNMETDTAEIRLMCTKTYLDNPRPNDGSITGPCESDGNEGSGGIKGGFVHQRMASKIARWYSRTMSKTKRMGMGLYVKYDGDPWTDSEALALSGVMISMEEPGWYSFGFEIRDKKCDVPCIGVEMVHDGGKKTWHSAATAIYCLMGSGQPLWDTVTGVNITL

SEQ ID NO: 71 - protein, 466 aa, synthetic construct
  REGION 1..466: note = synthetically-generated protein
MLPTTIQTLTLFLTSGGVLLSLYMSASLSYLLYSDMLLKFSRTEVTAPMMPLDCANASNVQAVNRSATKGVTPLLPEPEWTYPRLSCQGSTFQKALLISPHRFGETRGNSAPLIIREPFVACGPKECKHFALTHYAAQPGGYYNGTRGDRNKLRHLISVKLGKVPTVENSMFHMTAWSGSACHDGREWIYIGVDGPDSNALLKIKYGEAYTDTYHSYANNILRTQESACNCIRGDCYLMITDGPASGISECRFLKIREGRIIKEIFPTGRVEHTEECTCGFASNKTIECACRDNNYTAKRPFVKLNVETDTAEIKLMCTKTYLDTPRPNDGSITGPCESDGKEGSGGIKGGFVHQRMASKIGRWYSRTMSKTQRMGMGLYVKYDGDPWTDSDALALSGVMVSMEEPGWYSFGFEVKDKKCDVPCIGMEMVHDGGKTTWHSAATAVYCLMGSGQLLWDTVTGVNMTL

SEQ ID NO: 72 - protein, 466 aa, synthetic construct; identical to SEQ ID NO: 68
  REGION 1..466: note = synthetically-generated protein

SEQ ID NO: 73 - protein, 466 aa, synthetic construct
  REGION 1..466: note = synthetically-generated protein
MLSSTIQTLTLLLTSGGVLLSLYVSALLSYLLYSDMLLKFSRTEVTAPMMPLDCANASNVQAVNRSVTKGVTPLLPEPEWMYPRLSCPGSTFQRALLISPHRFGEIKGNSAPLIIREPFVACGPKECKHFALTHYTAQPGGYYNGTRGDRNKLRHLVSVKLGKIPTVENSMFHMAAWSGSACHDGKEWTYIGVDGPDNNALLKIKYGETYTDTYHSYANNILRTQESACNCIGGNCYLMITDGSASGVSECRFLKIREGRIVKEIFPTGRTQHTEECTCGFANNKTIECACRDNRYTAKRPFVKLNVEIDTAEIRLMCTETYLDTPRPDDGSITGPCESDGKEGSGGIKGGFVHQRMESKIGRWYSRTMSKTKRMGMGLYVKYNGDPWADSDALALSGVMISMEEPGWYSFGFEIRDKKCDVPCIGVEMVHDGGKETWHSAATAVYCLMGSGQPLWDTVTGVDMAL

SEQ ID NO: 74 - protein, 466 aa, synthetic construct
  REGION 1..466: note = synthetically-generated protein
MLPTTIQTLTLFLTTGGVLLSLYMSASLSYLLYLDILLKFPSTEITAPTMPLDCANASNAQAVNRSATKGVTLLLPEPEWTYPRLSCQGSTFQKALLISSHRFGETKGNSAPLIMREPFIACGPNECKHFALTHYATQPGGYYNGTREDRNNLRHLISVKLGKVPTVENSMFHMTAWSGSACHDGREWIYIGVDGPDNNALLKVKYGEAYTDTYHSYANKILRTQESACNCIRGDCYLMITDGPASGVSECRFLKIREGRIMKEIFPTGRVEHTEECTCGFASNKTIECACRDIPYTAKRPFVKLNVETDTAEIKLMCTKTYLDNPRPNDGSITGPCESDGDEGSGGIKGGLVHQRMASKIARWYSRTMSKTERKGMGLYVKYDGDPWTDSDALALSGVMVPMEEPGWYSFGFEIKDRKCDVPCIGLEMVHDGGKKTWHSAATAIYCLMGSGRLLWDTVTGVNITL

SEQ ID NO: 75 - protein, 548 aa, synthetic construct
  REGION 1..548: note = synthetically-generated protein
  REGION 180..181: note = misc_feature - X can be any naturally occurring amino acid
MMKAILVLLTFTAAYADTCIGYHANNSTDTVDTVLEKNVTVTHSVNLLEDHNGKLCKLGAPLLGKCNIAGWILGNPECESLTASWSYIVETSNSDNGTCYPGDFDYEELREQLSSVSSFERFEIFPKSSWPNHTGVTAACHNGSFYRNLIWLVKKGKENSYPKLSKSYNNKKEVLVLWGXXIHHPSTDQQLYQNAAYVFVGSSYSRKFPEIARPKVRDQGRMNYYWTLEPGDTITFEATGNLVAPRYAFALRGGSGIISDAPVHDCDTCQTPGAINTSLTSLPFQNVHPVTIGECPKYVKSTKLRMATGLRNIPSIQSRGLFGAIAGFIEGGWTGMIDGWYGYHHQNEQGSGYAADQKSTQNAIDGITNKVNSVIEKMNTQFTAVGKEFNLERRIENLNKKVDDGFLDIWTYNAELLVLLENERTLDFHDSNVKNLYEKVRSQLKNNAKEIGNGCFEFYHKCDNCMESVKNGTYDYPKYSEESKLNREEIDGVKLESRIYQILAIYSTVASSLVLLVSLGAISFWMCSNGSLQCRICIKNRDMRKNTL

SEQ ID NO: 76 - protein, 566 aa, synthetic construct
  REGION 1..566: note = synthetically-generated protein
MKAILVVLLYTFTTANADTLCIGYHANNSTDTVDTVLEKNVTVTHSVNLLENRHNGKLCKLRGVAPLHLGKCNIAGWLLGNPECESLSTASSWSYIVETSNSDNGTCYPGDFINYEELREQLSSVSSFERFEIFPKTSSWPNHDTNRGVTAACPHAGTNSFYRNLIWLVKKENSYPKINKSYINNKEKEVLVLWAIHHPSTSADQQSLYKNADAYVFVGSSRYSRKFEPEIATRPKVRDQAGRMNYYWTLLDQGDTITFEATGNLVAPRYAFALKRNSGSGIIISDTSVHDCDTTCQTPNGAINTSLPFQNIHPVTIGECPKYVKSTKLRMATGLRNIPSVQSRGLFGAIAGFIEGGWTGMIDGWYGYHHRNEQGSGYAADLKSTQNAIDGITNKVNSVIEKMNTQFTAVGKEFSHLERRIENLNKKVDDGFLDIWTYNAELLVLLENERTLDYHDSNVKNLYEKVRSQLKNNAKEVGNGCFEFYHKCDDTCMESVKNGTYDYPKYSEEAKLNREEIDGVKLESTRIYQILAIYSTVASSLVLVVSLGAISFWMCSNGSLQCKICI

SEQ ID NO: 77 - protein, 565 aa, synthetic construct
  REGION 1..565: note = synthetically-generated protein
MKVKLLILLCTFTATYADTICIGYHANNSTETVDTVLEKNVAVTHSVNLLEDSHNGKLCLLKGIAPLQLGNCSVAGWILGNPECESLISKKSWSYIVETPNPENGACYPGEFADYEELREQLSSVSSFKRFEIFPKESSWPNHTVTGVSASCSHNGERSFYRNLIWLTVKNGLYPNLSKSYENDKGKEVLILWGVHHPSNIGDQRTLYHTENAYVSVVSSHYSRRFTPEITKRPKVRDQEGRINYYWTLLEPGDTIIFEANGNLIAPWYAFALSRGLGSGIITSNAPMDECDAKCQTPQGAINSSLPFQNVHPVTIGECPKYVRSAKLRMVTGLRNIPSIQSRGLFGAIVGFIEGGWTGMVDGWYGYHHQNGQGSGYAADQESTQNAINGITNKVNSIIEKMNTQFTAVGKEFNKLERRMENLNKKVDDGLLDVWTYNAEMLVLLENERTLDFHDSNVKSLYEKVKSQLKNNAKEIGNGCFEFYHKCNNECMESVRNGTYDYPKYYEESKLNREKIDGVKLDSMGVYRILAIYSTAASSLVLLVSLGAISFWVCSNGSLQCRICI

SEQ ID NO: 78 - protein, 566 aa, synthetic construct
  REGION 1..566: note = synthetically-generated protein
MEAKLFVLFCAFTALKADTICVGYHANNSTDTVDTILEKNVTVTHSVNLLEDKHNGKLCKLGGIAPLHLGKCNIAGWILGNPECELLISKESWSYIVETSSSDNGTCYPGDFIDYEELREQLSTVSSFERFEIFPKASSWPNHDSNKGVTAACPHAGAKSFYKNLIWLVKKGNSYPKLSKSYINDKGKEVLVLWGIHHPSTSADQQSLYQNADAYVFVGTSRYSKKFKPEIAIRPKVRDQEGRMNYYWTLVEPGDKITFEATGNLVVPRYAFAMERNAGSGIIISDTPVHDCNTTCQTPKGAINTSLPFQNIHPITIGKCPKYVKSTKLRLATGLRNVPSIQSRGLFGAIAGFLEGGWTGMVNGWYGYHHQNEQGSGYAADQKSTQIAIDGISNKVNSVIEKMNIQFTSVGKEFNHLEKRIENLNKKVDDGFLDVWTYNAELLILLENERTLDFHDFNVKNLYEKVKSQLRNNAKEIGNGCFEFYHKCDNECMESVKNGTYNYPKYSEESKLNREEIDGVKLESMGVYRILSIYSTVASSLVLLVSLGAVSFWMCSNGSLQCRVCI

SEQ ID NO: 79 - protein, 566 aa, synthetic construct
  REGION 1..566: note = synthetically-generated protein
MKAILVVLLYTFTTANADTLCIGYHANNSTDTVDTVLEKNVTVTHSVNLLEDSHNGKLCKLRGVAPLHLGKCNIAGWLLGNPECESLSTASSWSYIVETSNSDNGTCYPGDFINYEELREQLSSVSSFERFEIFPKTSSWPNHDTNRGVTAACPHAGTNSFYRNLIWLVKKGNSYPKLSKSYINNKEKEVLVLWAIHHPSTSADQQSLYQNADAYVFVGSSRYSRKFEPEIATRPKVRDQAGRMNYYWTLVEPGDKITFEATGNLVVPRYAFALKRNSGSGIIISDTSVHDCDTTCQTPNGAINTSLPFQNIHPVTIGECPKYVKSTKLRMATGLRNIPSIQSRGLFGAIAGFIEGGWTGMIDGWYGYHHQNEQGSGYAADLKSTQNAIDGITNKVNSVIEKMNTQFTAVGKEFNKLERRMENLNKKVDDGFLDIWTYNAELLVLLENERTLDYHDSNVKNLYEKVRSQLKNNAKEIGNGCFEFYHKCNNECMESVKNGTYDYPKYSEEAKLNREEIDGVKLESTRIYQILAIYSTVASSLVLLVSLGAISFWMCSNGSLQCRICI

SEQ ID NO: 80 - protein, 565 aa, synthetic construct
  REGION 1..565: note = synthetically-generated protein
MKVKLLILLCTFTATYADTICIGYHANNSTDTVDTILEKNVTVTHSVNLLENRHNGKLCLLKGIAPLQLGNCSVAGWILGNPECESLISKKSWSYIVETPNPENGACYPGEFADYEELREQLSTVSSFERFEIFPKESSWPNHTVTGVSASCSHNGERSFYRNLIWLTVKNGLYPNLSKSYENDKGKEVLILWGVHHPSNIGDQRTLYHTENAYVSVVSSHYSRRFTPEITKRPKVRDQEGRINYYWTLLEPGDTIIFEANGNLIAPWYAFALSRGLGSGIITSNAPMDECDAKCQTPQGAINSSLPFQNVHPVTIGECPKYVRSAKLRMVTGLRNVPSIQSRGLLGAIAGFIEGGWTGMVDGWYGYHHQNGQGSGYAADQESTQNAINGITNKVNSIIEKMNIQFTSVGKEFNHLEKRIENLNKKVDDGFLDVWTYNAELLILLENERTLDFHDSNVKSLYEKVKSQLKNNAKEVGNGCFEFYHKCDDTCMESVKNGTYNYPKYSEESKLNREKIDGVKLDSMGVYRILAIYSTVASSLVLVVSLGAISFWMCSNGSLQCRVCI

SEQ ID NO: 81 - protein, 566 aa, synthetic construct
  REGION 1..566: note = synthetically-generated protein
MEAKLFVLFCAFTALKADTICVGYHANNSTETVDTVLEKNVAVTHSVNLLEDKHNGKLCKLGGIAPLHLGKCNIAGWILGNPECELLISKESWSYIVEAPNSDNGACYPGQFADYEELREHLSSVSSFEKFEIFPKASSWPNHDSNKGVTAACPYAGANSFYRNLLWIVKKGNSYPKINKSYINNKGKEVLVLWGIHHPPTSTDQQSLYKNADAYVFVGTSRYSKKFKPEIAIRPKVRDQEGRMNYYWTLLDQGDTITFEATGNLVAPRYAFAMERNAGSGIIISDTPVHDCNTTCQTPKGAINSNLPFQNVHPITIGECPKYVRSTKLRMVTGLRNIPSVQSRGLFGAIAGFLEGGWTGMVNGWYGYHHQNDQGSGYAADQKSTQIAIDGISNKVNSVIEKMNIQFTAVGKEFSHLERRIENLNKKVDDGLLDVWTYNAEMLVLLENERTLDFHDFNVKNLYEKVKSQLRNNAKEIGNGCFEFYHKCDNTCMESVRNGTYDYPKYYEESKLNREEIDGVKLESMGVYQILAIYSTAASSLVLLVSLGAVSFWMCSNGSLQCKICI

SEQ ID NO: 82 - protein, 571 aa, synthetic construct
  REGION 1..571: note = synthetically-generated protein
MKTIIAFSCILCLIFAQKLPGSDNNSMATLCLGHHAVPNGTLVKTITDDQIEVTNATELVQSSSTGRICNSPGHQILDGKNCTLIDALLGDPHCDDFQNKWDLFVERSTAYSGNCYPYYVPDYASLREQLSLVASSGTLEFTQESFNWTGVAQDGSSYACRRGSVNNSFFSRLNWLYLNYKYPALNVTMPNNDKFDKLYIWGVHHPGTDKDQTNLYVQASGRVVSTKRSQQTVIPNIGSRPWVRGVSSIISIYWTIVKPGDILLINSTGNLIAPRGYFKIQSGKSSGIMRSDAPIDCNSECITPNGSIPNDKPFQNVNRITYGACPRYVKQNTLKLATGMRNVPEKQTRGIFGAIAGFIENGWEGMVDGWYGFRHQNSEGTGQAADLKSTQAAINQITGKLNRVIKKTNEKFHQIEKEFSEVEGRIQDLEKYVEDTKIDLWSYNAELLVALENQHTIDLTDSEMNKLFERTRKQLRENAEDMGNGCFKIYHKCDNACIGSIRNGTYDHDVYRDEALNNRFQIKGVQLKSGYKDWILWISFAISCFLLCVVLLGFISMWACQKGNIRCNICI

SEQ ID NO: 83 - protein, 566 aa, synthetic construct
  REGION 1..566: note = synthetically-generated protein
MKTIIAFSCILCLIFAQKLPGSDNSTATLCLGHHAVPNGTMVKTITDDQVEVTNATELVQSSSTGRICNSPHQILDGKNCTLIDSLLGDPHCDDFQNKEWDLFVERSKAYSNCYPYYVPDYATLRSLVASSGNLEFTQESFNWTGVAQDGSSYACRRGSVNSFFSRLNWLYNLNYKYPEQNVTMPNNDKFDKLYIWGVHHPGTDKDQTNLYVQASGRVIVSTKRSQQTIIPNIGSRPWVRGVSSIISIHWTIVKPGDILLINSTGNLIAPRGYFKIQNGKSSIMRSDAHIDECNSECITPNGSISNDKPFQNVNKITYGACPRYIKQNTLKLATGMRNIPEKQTRGIFGAIAGFIENGWEGMVNGWYGFRHQNSEGTGQAADLKSTQAAINQITGKLNRVIKKTNEKFHQIEKEFSEVEGRIQDLEKYVEDTKIDIWSYNAELLVALENQHTIDLTDSEMSKLFERTRRQLRENAEDIGNGCFKIYHKCDNSCMESIRNGTYDHDIYRNEALNNRFQIKGVQLKSGYKDWILWISFAISCFLLCVVLLGFIMWACQRGNIRCNICV

SEQ ID NO: 84 - protein, 566 aa, synthetic construct
  REGION 1..566: note = synthetically-generated protein
MKTIIALSYILCLVFAQKLPGNDNNMATLCLGHHAVPNGTIVKTITNDQIEVTNATELVQSFSTGEICNSPHQILDGENCTLIDALLGDPQCDGFQNNKWDLFVERSKAHSNCYPYDVPDYASLRSLVASSGTLEFNNESFNWTGVTQNGGSSACKRGPNNSFFSRLNWLTHLNFKYPALEVTMPNNEQFDKLYIWGVHHPATDKDQISLYAQAAGRIIVSTKRSQQAVIPNIGSRPRVRDIPSRISIYWTIVRPGDILLIKSTGNLIAPRGYFKIRSGKSSIMRSDAPIGKCNSACITPNGSIPNDKPFQNVNRITYGACPKYVKQNTLKLATGMRNIPERQTRGIFGAKAGFIENGWEGMVDGWYGFRHQNSEGRGQAADLKSTQAAIDQINGKLNRLIGKTNEKFHQIEKEFSEIEGRIQDLEKYIEDTKIDLWSYNAELLIALENQHTIDLADSEMNKLFEKTKKQLRENAEDMGNGCLKIYHKCDNACIGSIRNGTYDHDVYRDEALNNRFQIKGVELKSEYKDWILWISFAMSCFLLCVALLGFIMWACQKGNIKCNICI

SEQ ID NO: 85 - protein, 566 aa, synthetic construct
  REGION 1..566: note = synthetically-generated protein
MKAIIAFSCILCQISAQKLPGSDNSMATLCLGHHAVPNGTLVKTITDDQIEVTNATELVQSTSKGEICSSPHQILDGKNCTLIDALLGDPHCDDFQNKKWDLFVERSTAYSNCYPYYVPDYASLRSLIASSGTLEFTQESFDWTGVAQNGSSYACRRGSVKSFFSRLNWLHNLNYKYPALNVTMPNNDNFDKLYIWGVHHPSTDSDQTSLYVQASGRVTVSTKRSQQTVIPNIGSRPWIRGVSSIISIYWTIVKPGDILIINSNGNLIAPRGYFKIQSGKSSIMRSDAPIGNCNSECITPNGSIPNDRPFQNVNRITYGACPRYVKQNTLKLATGMRNVPEKQTRGILGAIAGFIENGWEGMIDGWYGFRHHNSEGTGQAADIKSTQAAINQINGKLNRVIEKTNEKFHQIEKEFSGVEGRIQDLERYVEDTKIDLWSYNAELLVAMENQHTIDLTDSEMNKLFERTRKQLRENAEDMGNGCFKIYHKCDNTCIGSIRNGTYNHDVYRDEAVNNRFQIKGVQLKLGYKDWILWISFATSCFLLCAVLLGFIMWACQKGNIRCNICI

SEQ ID NO: 86 - protein, 566 aa, synthetic construct
  REGION 1..566: note = synthetically-generated protein
MKTIIAFSCILCLIFAQKLPGSDNSMATLCLGHHAVPNGTLVKTITDDQIEVTNATELVQSSSTGRICNSPHQILDGKNCTLIDALLGDPHCDDFQNKEWDLFVERSTAYSNCYPYYVPDYASLRSLVASSGTLEFTQESFNWTGVAQDGSSYACRRGSVNSFFSRLNWLYNLNYKYPEQNVTMPNNDKFDKLYIWGVHHPGTDKDQTNLYVQASGRVIVSTKRSQQTVIPNIGSRPWVRGVSSIISIYWTIVKPGDILLINSTGNLIAPRGYFKIQSGKSSIMRSDAHIDECNSECITPNGSIPNDKPFQNVNRITYGACPRYVKQNTLKLATGMRNVPEKQTRGIFGAIAGFIENGWEGMVDGWYGFRHQNSEGTGQAADLKSTQAAINQITGKLNRVIKKTNEKFHQIEKEFSEVEGRIQDLEKYVEDTKIDLWSYNAELLVALENQHTIDLTDSEMNKLFERTRKQLRENAEDMGNGCFKIYHKCDNACIGSIRNGTYDHDVYRDEALNNRFQIKGVQLKSGYKDWILWISFAISCFLLCVVLLGFIMWACQKGNIRCNICI

SEQ ID NO: 87 - protein, 566 aa, synthetic construct
  REGION 1..566: note = synthetically-generated protein
MKTIIALSYILCLVFAQKLPGNDNNMATLCLGHHAVPNGTIVKTITNDQIEVTNATELVQSTSKGEICSSPHQILDGENCTLIDALLGDPHCDDFQNKKWDLFVERSKAHSNCYPYYVPDYATLRSLVASSGNLEFTQESFNWTGVTQDGASSACKRRSSKSFFSRLNWLHNLNYKYPALNVTMPNNDNFDKLYIWGVHHPSTDKDQTSLYIQASGRVTVSTKRSQQAVIPNIGSRPRVRDIPSRISIYWTIVRPGDILLINSNGNLIAPRGYFKIRSGKSSIMRSDAPIGNCNSECITPNGSISNDKPFQNVNKITYGACPRYIKQNTLKLATGMRNIPEKQTRGIFGAKAGFIENGWEGMVNGWYGFRHQNSEGRGQAADLKSTQAAIDQINGKLNRLIGKTNEKFHQIEKEFSEIEGRIQDLERYVEDTKIDIWSYNAELLVAMENQHTIDLTDSEMSKLFERTRRQLRENAEDMGNGCLKIYHKCDNSCMESIRNGTYDHDIYRNEALNNRFQIKGVELKSEYKDWILWISFATSCFLLCAVLLGFIMWACQKGNIKCNICI

SEQ ID NO: 88 - protein, 566 aa, synthetic construct
  REGION 1..566: note = synthetically-generated protein
MKAIIAFSCILCQIFAQKLPGNDNSTATLCLGHHAVSNGTLVKTITDDQVEVTNATELVQNFSMGKICKNPHRILDGANCTLIDSLLGDPHCDGFQNEKWDLFIERSKAFSNCYPYDVPDYASLRSLIASSGTLEFNNESFNWTGVTQNGGSSACKRGPNNSFFSRLNWLTHLNFKYPALEVTMPNNEQFDKLYIWGVHHPATDKDQISLYAQAAGRIIVSTKRSQQTIIPNIGSRPWIRGVSSIISIHWTIVKPGDMLLINSTGNIIAPRGYFKIQTGKSSVMRSDAPIGKCNSACITPNGSIPNDRPFQNVNKITYGACPKYVKQNTLKLATGMRNIPERQTRGIFGAIAGFIENGWEGMIDGWYGFRHHNSEGTGQAADIKSTQAAINQINGKLNRVIEKTNEKFHQIEKEFLEVEGRIQDIEKYIEDTKIDLWSYNAELLIALENQHTIDLADSEMNKLFEKTKKQLRENAEDIGNGCFKIYHKCDNTCIGSIRNGTYNHDVYRDEAVNNRFQIKGVQLKLGYKDWILWISFAMSCFLLCVALLGFIMWACQRGNIRCNICV

SEQ ID NO: 89 - protein, 465 aa, synthetic construct
  REGION 1..465: note = synthetically-generated protein
MNTNQRIITIGTVCMIVGIISLLLQIGNIVSLWISHSIQTGNENHTHECNQSVITYENNTWVNQTYVNISNTNIAQVTSVTSIILAGNSSLCPVSGWAIYSKDNSIRIGSKGDIFVIREPFISCSLECRTFFLTQGALLNDKHSNGTVKDRSPYRTLMSCPIGEAPSPYNSRFESVAWSASACHDGMGWLTIGISGPDNGAVAVLKYNGIITDTIKSWRNILRTQESECVCNGSCFTVMTDGPSNGQASYKIFKEKGKIIKSVELDAPNYHYEECSCYPDTGKVVCVCRDNWHASNRPWVSFNQNLDYQIGYICSGVFGDNPRSNDGKGNCGPVLSNGANGVKGFSFRYGNGVWIGRTKSISSRSGFEMIWDPNGWTETDSSFSIKQDIIALNDWSGYSGSFVQHPELTGMNCIRPCFWVELIRGQPKENTIWTSGSSISFCGVNSETASWSWPDGADLPFTIDK

SEQ ID NO: 90 - protein, 469 aa, synthetic construct
  REGION 1..469: note = synthetically-generated protein
MNTNQRIITIGTVCMIVGIISLLLQIGNIVSLWISHSIQTGWENHTEMCNQSVITYVNNTWVNRTYVNISNIKIATIQDVTSIILAGNSSLCPVSGWAVYSKDNSIRIGSKGDVFVMREPFISCSQLECRTFFLTQGALLNDKHSNGTVKDRSPHRTLMSCPVGEVPSPYNSKFESVAWSASACHDGMGWLTIGISGPDDGAVAVLKYNGIITDTIKSWRNKILRTQESECVCMNGSCFTVLTDGPSNGQASYKIFKVEKGKIIKSIELDAPNYHYEECSCYPDTGKVMCVCRDNWHASNRPWVSFNQNLDYQIGYICSGVFGDNPRSNDGKGNCGPVLSNGANGVKGFSYRYGNGVWIGRTKSINSRSGFEMIWDPNGWTETDSSFSMKQDIIALNDWSGYSGSFVQHPELTGMNCIRPCFWVELIRGQPKESTIWASGSSISFCGVNSETASWSWPDGANLPFTIDK

SEQ ID NO: 91 - protein, 469 aa, synthetic construct
  REGION 1..469: note = synthetically-generated protein
MNTNQKIITIGSVCMTIGMANLILQIGNIISIWISHSIQLGNQNQIETCNQSVITYENNTWVNQTYVNISNTNFAAGQSVVSVKLAGNSSLCPVSGWAIYSKDNSVRIGSKGDVFVIREPFISCSPLECRTFFLTQGTLLNDKHSNGTIKDRSPYRTLMSCPIGEVPSPYNSRFESVAWSASACHDGINWLTIGISGPDSGAVAVLKYNGVITDTIKSWRNNILRTQESECVCINGSCFTIMTDGPSDGQASYKIFRIEKGKIVKSVEMNAPNYHYEECSCYPDSSEITCVCRDNWHASNRPWVSFDQNLDYQIGYICSGIFGDNPRPNDKTGSCGPVSSNGANGVKGFSFRYGNGVWIGRTKSISSRNGFEMIWDPNGWTGTDNNFSIKQDIVGINEWSGYSGSFVQHPELTGLDCIRPCFWVELIRGRPKENTIWTSGSSISFCGVNSDTVGWSWPDGAELPFTIDK

SEQ ID NO: 92 - protein, 469 aa, synthetic construct
  REGION 1..469: note = synthetically-generated protein
MNPNQKIITIGSICMTIGIASLILQIGNIVSLWVSHSIQTRWENHTEVCNQNVITYVNNTLVNRTYVNISNTNIATIQDVTSIMLAGNSSLCPISGWAIYSKDNSIRIGSKGDIFVIREPFISCSHLECRTFFLTQGALLNDRHSNGTVKDRSPYRTLMSCPIGEAPSPYNSRFESVAWSASACHDGTSWLTIGISGPDNGAVAVLKYNDIITDTIKSWRKNILRTQESECACVNGSCFTVMTDGPSNGQASYKIFKIEKGKVVKSVELNAPNYHYEECSCYPDTGKVVCVCRDNWHGSNRPWVSFNQNLEYQIGYICSGVLGDNPRPNDRTGSCGPVFSNGANGVKGFSFKYGNGVWIGRTKSTSSRSGFEMIWDPDGWTRTDDKFSVKQDIIALTDWSGYSGSFVQHPELTGLDCMRPCFWVELIRGQPKENTIWASGSSISFCGVDSETASWSWPDGADLPFTIDK

SEQ ID NO: 93 - protein, 469 aa, synthetic construct
  REGION 1..469: note = synthetically-generated protein
MNTNQRIITIGTVCMIVGIISLLLQIGNIVSLWISHSIQTGWENHTEMCNQSVITYENNTWVNQTYVNISNIKIATIQDVTSIILAGNSSLCPVSGWAIYSKDNSIRIGSKGDIFVIREPFISCSQLECRTFFLTQGALLNDKHSNGTVKDRSPYRTLMSCPIGEAPSPYNSRFESVAWSASACHDGMGWLTIGISGPDNGAVAVLKYNGIITDTIKSWRNKILRTQESECVCMNGSCFTVLTDGPSNGQASYKIFKVEKGKIIKSIELDAPNYHYEECSCYPDTGKVMCVCRDNWHASNRPWVSFNQNLDYQIGYICSGVFGDNPRSNDGKGNCGPVLSNGANGVKGFSYRYGNGVWIGRTKSINSRSGFEMIWDPNGWTETDSSFSMKQDIIALTDWSGYSGSFVQHPELTGMNCIRPCFWVELIRGQPKESTIWASGSSISFCGVNSETASWSWPDGADLPFTIDK

SEQ ID NO: 94 - protein, 469 aa, synthetic construct
  REGION 1..469: note = synthetically-generated protein
MNPNQKIITIGSVCMTIGMANLILQIGNIISIWISHSIQLGNQNQIETCNQSVITYVNNTWVNRTYVNISNTNFAAGQSVVSVKLAGNSSLCPISGWAIYSKDNSVRIGSKGDVFVIREPFISCSHLECRTFFLTQGSLLNDKHSNGTIKDRSPYRTLMSCPIGEVPSPYNSRFETVAWSASACHDGINWLTIGISGPDSGAVAVLKYNDIITDTIKSWRNNILRTQESECACVNGSCFTVMTDGPSDGQASYKIFRIEKGKIVKSVEMNAPNYHYEECSCYPDSSEITCVCRDNWHGSNRPWVSFNQNLEYQIGYICSGIFGDNPRPNDKTGSCGPVSSNGANGVKGFSFKYGNGVWIGRTKSISSRNGFEMIWDPNGWTGTDNNFSIKQDIIALNDWSGYSGSFVQHPELTGLDCIRPCFWVELIRGRPKENTIWTSGSSISFCGVNSDTVGWSWPDGAELPFTIDK

SEQ ID NO: 95 - protein, 469 aa, synthetic construct
  REGION 1..469: note = synthetically-generated protein
MNTNQKIITIGSICMTIGIASLILQIGNIISIWVSHSIQTRWENHTEVCNQNVITYVNNTWVNQTYVNISNTNIATIQDVTPIILAGNSPLCPVSGWAVYSKDNSIRIGSKGDIFVMREPFISCSPLECRTFFLTQGALLNDRHSNGTVKDRSPHRTLMSCPVGEVPSPYNSKFESVAWSASACHDGTSWLTIGISGPDDGAVAVLKYNGVITDTIKSWRKNILRTQESECVCINGSCFTIMTDGPSNGQASYKIFKIEKGKVVKSVELNAPNYHYEECSCYPDTGKVVCVCRDNWHASNRPWVSFDQNLDYQIGYICSGVLGDNPRPNDRTGSCGPVFSNGANGVKGFSFRYGNGVWIGRTKSTSSRSGFEMIWDPDGWTRTDDKFSVKQDIVGINEWSGYSGSFIQHPELTGLDCMRPCFWVELIRGQPKENTIWASGSSISFCGVDSETASWSWPDGANLPFTIDK

SEQ ID NO: 96 - protein, 466 aa, synthetic construct
  REGION 1..466: note = synthetically-generated protein
MNPNQKIITIGSVSLIIATICFLMQIAILVTTVTLHFKQHDCNSPPNNQVMLCEPPTIIERNTEIVYLTNTTIEKEICPKLAEYRNWSKPQCNITGFAPFSKDNSIRLSAGGDIWVTREPYVSCDPDKCYQFALGQGTTLNNGHSNDTVHDRTPYRTLLMNELGVPFHLGTRQVCIAWSSSSCHDGKAWLHVCITGDDENATASFIYNGRLVDSIGSWSKNILRTQESECVCINGTCTVVMTDGSASGKADTKILFIEEGKIIHISTLSGSAQHVEECSCYPRYPGVRCVCRDNWKGSNRPIVDINVKDYSIVSSYVCSGLVGDTPRKNDSSSSCLDPNNEEGGHGVKGWAFDDGNDVWMGRTISEELRLGYETFKVIGWSKPNSKLQTNRQVIVERGNRSGYSGIFSVEGKSCINRCFYVELIRGRKEETKVWWTSNSIVVFCGTSGTYGTGSWPDGADINLMPI

SEQ ID NO: 97 - protein, 469 aa, synthetic construct
  REGION 1..469: note = synthetically-generated protein
MNPNQKIITIGSVSLTIATICFLMQIAILVTTVTLHFKQHDYNSPPNNQAMLCEPTIIERNTTEIVYLTNTTIEKEICPKLAEYRSWSKPQCNITGFAPFSRDNSIRLSAGGDIWVTREPYVSCDHDKCYQFALGQGTTLNNGHSNNTVHDRTPYRTLLMNELGVPFHLGTRQVCMAWSSSSCHDGRAWLHVCITGNDNNATASFIYDGRLVDSIGSWSKKILRTQESECVCINGICTVVMTDGSASEKADTKILFVEEGKIVHISTLSGSAQHVEECSCYPRFPGVRCVCRDNWKGSNRPIVDINVKNYSIVSSYVCSGLVGDTPRKSDSVSSSYCLDPNNEKGGHGVKGWAFDDGNDVWMGRTINETLRLGYETFKVIEGWSKANSKLQTNRQVIVEKGDRSGYSGIFSIEGKNCINRCFYVELIRGRKQETEVWWTSNSIVVFCGTSGTYGAGSWPDGADISLMPI

SEQ ID NO: 98 - protein, 469 aa, synthetic construct
  REGION 1..469: note = synthetically-generated protein
MNPNQKIITIGSISLTLAAMCFLMQIAILVTNVTLHFKQHNCDSSPNNHVMFCEPTIIERNITEIVYLTNITIEKEKCPKLAEYRNWSKPQCKITGFAPFSKDNSIRLSAGGAIWVTREPYVSCDPDKCYQFALGQGTTLNNRHSNDTIHDRTPYRTLLMSELGVPFHLGTRQVCIAWSSSSCYDGKAWLHVCITGDDKNATASFIYNGRLVDSIGSWSKNILRTQESECVCINGTCAVVMTDGSASGKADTKILFIEEGKIVHISPLLGSAQHVEECSCYPRYPGVRCVCRDNWRGSNRPIVDINVKDYSIVSSYVCSGLVGDTPRKDDKSSSSNCLNPNNEEGGHGVKGWAFDDGDDVWMGRTISEKLRSGYETFKVIEGWSKPNSKLQINRQVIVDRGNRSGYSGIFSVEGKSCINRCFYVELIRGRRQETRVWWTSNSIIVFCGTSGTYGSGSWPDGADINFMPI

SEQ ID NO: 99 - protein, 469 aa, synthetic construct
  REGION 1..469: note = synthetically-generated protein
MNPNQRIITIGSVSLIIATICFLMQVAILVTTVTLHFKQHDCNSSPNNQVMLCEPTIIERNKTEIVYLTNTTVEKEICPKPAEYRNWSKPQCNIAGFAPFSKDNSVRLSAGGDIWITREPYVSCDLDKCYQFALGHGTTLNNGHSNDTVHDRTPYRTLLMNELGIPFHLGTKQVCIAWSSSSCHDGKAWLHVCVTGHDENATASIIYNGRLVDSIGSWSQNILRTQESECVCINGTCTVVMTDGSASGRADTKILFIEEGKIIHISTLSGSAKHVEECSCYPRYPGVRCICRDNWKGSNRPVVDINVKDYSTVSSYVCSGLVGDTPRKNDSFSSSHCLDPNNEEGGHGVKGWAFDDGNDLWMGRTISEKSRLGYETFKVIKGWSKPNSKLQTNRQVIVGRGNRSGYSGIFSVEGKNCINRCFYVELIRGRKEETKVWWTSNSILVFCGTSGTYGTGSWPDGADINLMPI

SEQ ID NO: 100 - protein, 469 aa, synthetic construct
  REGION 1..469: note = synthetically-generated protein
MNPNQKIITIGSVSLIIATICFLMQIAILVTTVTLHFKQHDYNSPPNNQVMLCEPTIIERNKTEIVYLTNTTIEKEICPKLAEYRNWSKPQCNITGFAPFSKDNSIRLSAGGDIWVTREPYVSCDPDKCYQFALGQGTTLNNGHSNDTVHDRTPYRTLLMNELGVPFHLGTRQVCIAWSSSSCHDGKAWLHVCITGDDKNATASFIYNGRLVDSIGSWSKNILRTQESECVCINGTCTVVMTDGSASGKADTKILFIEEGKIIHISTLSGSAQHVEECSCYPRYPGVRCVCRDNWKGSNRPIVDINVKDYSIVSSYVCSGLVGDTPRKNDSFSSSHCLDPNNEEGGHGVKGWAFDDGNDVWMGRTINETLRLGYETFKVIEGWSKPNSKLQTNRQVIVEKGDRSGYSGIFSVEGKSCINRCFYVELIRGRKEETKVWWTSNSIVVFCGTSGTYGTGSWPDGADINLMPI

SEQ ID NO: 101 - protein, 469 aa, synthetic construct
  REGION 1..469: note = synthetically-generated protein
MNPNQRIITIGSVSLTIATICFLMQVAILVTTVTLHFKQHDCNSSPNNQVMFCEPTIIERNTTEIVYLTNTTVEKEICPKPAEYRNWSKPQCKITGFAPFSRDNSIRLSAGGAIWVTREPYVSCDLDKCYQFALGQGTTLNNRHSNDTIHDRTPYRTLLMNELGIPFHLGTKQVCIAWSSSSCYDGKAWLHVCITGNDNNATASFIYDGRLVDSIGSWSKKILRTQESECVCINGICTVVMTDGSASGRADTKILFVEEGKIVHISTLSGSAKHVEECSCYPRYPGVRCICRDNWKGSNRPVVDINVKNYSIVSSYVCSGLVGDTPRKSDSVSSSYCLDPNNEKGGHGVKGWAFDDGDDVWMGRTISEKSRLGYETFKVIKGWSKPNSKLQINRQVIVDRGNRSGYSGIFSVEGKNCINRCFYVELIRGRKQETEVWWTSNSIIVFCGTSGTYGSGSWPDGADINFMPI

SEQ ID NO: 102 - protein, 469 aa, synthetic construct
  REGION 1..469: note = synthetically-generated protein
MNSNQKIITIGSISLTLAAMCFLMQIAILVTNVTLHFNQCECHYPPNNQVILCEPTIIERNITEIVYLTNITIEKEKCPKLAEYRSWSKPQCNIAGFAPFSKDNSVRLSAGGDIWITREPYVSCDHDKCYQFALGHGTTLNNGHSNNTVHDRTPYRTLLMSELGVPFHLGTRQVCMAWSSSSCHDGKAWLHVCVTGHDENATASIIYNGRLVDSIGSWSQNILRTQESECVCINGTCAVVMTDGSASGKADTRILFIEEGKIVHISPLLGSAQHVEECSCYPRFPGVRCVCRDNWRGSNRPVVDINVKDYSTVSSYVCSGLVGDTPRKDDKSSSSNCLNPNNEEGGHGVKGWAFDDGNDLWMGRTISEKLRSGYETFKVIEGWSKANSKLQTNRQVIVGRGNRSGYSGIFSIEGKNCINRCFYVELIRGRRQETRVWWTSNSILVFCGTSGTYGAGSWPDGADISLMPI

SEQ ID NO: 103 - DNA, 1680 bp, synthetic construct
  misc_feature 1..1680: note = synthetically-generated coding sequence
  source 1..1680: mol_type = other DNA
atgaaggtgaagctgctggtgctgctgtgcacctttacagccacctacgccgacacaatctgtatcggctatcacgccaacaattccacagacaccgtggataccgtgctggagaagaacgtgacagtgacccactccgtgaacctgctggaggattctcacaatggcaagctgtgcctgctgaagggcatcgccccactgcagctgggcaactgctctgtggccggctggatcctgggcaatcccgagtgtgagctgctgatcagcaaggagtcttggagctacatcgtggagacaccaaaccccgagaatggcacctgctaccccggctttgccgactatgaggagctgagggagcagctgagcagcgtgagcagcttcgagcggttcgagatcttccctaaggagtcctcttggccaaaccacacagtgaccaagggcgtgtccgcctcttgtagccacaacggcagctccttctaccggaatctgctgtggctgaccggcaagaacggcctgtaccctaatctgtccaagtcttatgccaacaataaggagaaggaggtgctggtgctgtggggagtgcaccacccacctaacatcggcgatcagctgtaccacacagagaatgcctatgtgagcgtggtgtctagccactactcccggtttacccccgagatcgccaagaggcctaaggtgcgcgaccaggagggcagaatcaactactattggacactgctggagcccggcgataccatcatcttcgaggccaacggcaatctgatcgcccctagatatgcctttgccctgtccaggggattcggaagcggaatcatctccaatgcccctatggacgagtgcgatgccaagtgtcagacaccacagggcgccatcaactcctctctgccatttcagaatgtgcaccccgtgacaatcggcgagtgtcctaagtacgtgcggagcgccaagctgagaatggtgaccggcctgcggaacatcccaagcatccagtccagaggcctgtttggagcaatcgcaggcttcatcgagggaggatggaccggaatggtggacggctggtacggctatcaccaccagaatgagcagggctctggctatgccgccgatcagaagagcacacagaacgccatcaatggcatcaccaacaaggtcaattccgtgatcgagaagatgaacacacagtttaccgccgtgggcaaggagttcaataagctggagcggagaatggagaacctgaataagaaggtggacgatggctttctggacatctggacatacaacgccgagctgctggtgctgctggagaatgagaggaccctggacttccacgattccaacgtgaagaatctgtatgagaaggtgaagtctcagctgaagaacaatgccaaggagatcggcaacggctgcttcgagttttaccacaagtgcaacgacgagtgtatggagagcgtgaagaatggcacatacgattatcccaagtattctgaggagagcaagctgaatagggagaagatcgatggcgtgaagctggagagcatgggcgtgtaccagatcctggccatctattccaccgtggcaagctccctggtgctgctggtgtctctgggcgccatcagcttctggatgtgctccaacggctctctgcagtgccgcatctgtatc

SEQ ID NO: 104 - DNA, 1695 bp, synthetic construct
  misc_feature 1..1695: note = synthetically-generated coding sequence
  source 1..1695: mol_type = other DNA
atgaaggtgaagctgctggtgctgctgtgcaccttcacagccacctacgccgacacaatctgtatcggctatcacgccaacaatagcacagacaccgtggataccgtgctggagaagaacgtgacagtgacccactctgtgaatctgctggagaacagccacaatggcaagctgtgcctgctgaagggcatcgccccactgcagctgggaaactgcagcgtggcaggatggatcctgggaaatccagagtgtgagctgctgatctccaaggagtcttggagctacatcgtggagaagccaaaccccgagaatggcacatgctaccccggccacttcgccgactatgaggagctgagggagcagctgagctccgtgtctagcctggagcggttcgagatctttcctaaggagtcctcttggccaaaccacacagtgaccggcgtgtccgcctcttgtagccacaacggcgagagctccttttacaggaatctgctgtggctgaccggcaagaacggcctgtaccctaatctgtccaagtcttatgccaacaataaggagaaggaggtgctggtgctgtggggagtgcaccacccacctaacatcggcgatcagcgcgccctgtaccacacagagaatgcctacgtgagcgtggtgtctagccactactctcggaagttcacccccgagatcgccaagaggcctaaggtgcgcgaccaggagggcagaatcaactactattggacactgctggagcccggcgataccatcatctttgaggccaacggcaatctgatcgcccctagatatgccttcgccctgagcaggggatttggatccggcatcatcaactctaatgcccctatggacaagtgcgatgccaagtgtcagaccccacagggcgccatcaactcctctctgccattccagaatgtgcaccccgtgacaatcggcgagtgtcctaagtacgtgcggagcgccaagctgagaatggtgaccggcctgcggaacatcccaagcgtgcagtccagaggactgttcggagcaatcgcaggctttatcgagggaggctggacaggcatgatcgacggctggtacggctatcaccaccagaatgagcagggcagcggctatgccgccgatcagaagtccacacagaacgccatcaatggcatcaccaacaaggtcaattccgtgatcgagaagatgaacatccagttcaccgccgtgggcaaggagtttaataagctggagcggagaatggagaacctgaataagaaggtggacgatggcttcatcgatatctggacatacaacgccgagctgctggtgctgctggagaatgagcggaccctggactttcacgattctaacgtgaagaatctgtatgagaaggtgaagagccagctgaagaacaatgccaaggaagtgggcaacggctgcttcgagttttaccacaagtgcaacgacgagtgtatggagtccgtgaagaatgagacctacgattatcccaagtattctgaggagagcaagctgaatagggagaagatcgacggcgtgaagctggattccatgggcgtgtaccagatcctgacaatctattctaccgtggccagctccctggtgctgctggtgagcctgggagccatctccttttggatgtgctccaacggctctctgcagtgcaagatctgtatc

SEQ ID NO: 105 - DNA, 1698 bp, synthetic construct
  misc_feature 1..1698: note = synthetically-generated coding sequence
  source 1..1698: mol_type = other DNA
atgaaggccatcctggtggtgctgctgtacacctttgccacagccaacgccgacaccctgtgcatcggctatcacgccaacaatagcaccgacacagtggatacagtgctggagaagaatgtgaccgtgacacactccgtgaacctgctggaggataagcacaatggcaagctgtgcaagctgaggggagtggcacctctgcacctgggcaagtgcaacatcgccggctggatcctgggcaatccagagtgtgagtccctgtctaccgccagctcctggtcctacatcgtggagacctctagctccgacaacggcacatgctaccctggcgactttatcgattatgaggagctgagggagcagctgtctagcgtgagcagcttcgagcggttcgagatcttccccaagaccagctcctggcctaaccacgatagcaataagggagtgacagcagcatgtccacacgcaggcgccaagtccttctacaagaacctgatctggctggtgaagaagggcaattcttaccccaagctgagcaagtcctatatcaacgacaagggcaaggaggtgctggtgctgtggggcatccaccacccatctaccagcgccgaccagcagtccctgtaccagaatgccgatgcctacgtgttcgtgggcacatcccggtactctaagaagttcaagccagagatcgccatccggcccaaggtgagagaccaggagggcagaatgaactactattggaccctggtggagccaggcgataagatcacctttgaggcaacaggaaacctggtggtgcccagatatgccttcgccatggagagaaatgccggctccggcatcatcatctctgacacccccgtgcacgattgcaacaccacatgtcagacccctaagggcgccatcaacacatctctgcctttccagaatatccacccaatcacaatcggcaagtgccccaagtacgtgaagagcaccaagctgaggctggccacaggcctgcgcaatgtgcctagcatccagtccaggggactgtttggagcaatcgcaggcttcatcgagggaggatggaccggaatggtggatggatggtacggctatcaccaccagaacgagcagggctctggctatgccgccgacctgaagagcacccagaatgccatcgataagatcacaaacaaggtcaatagcgtgatcgagaagatgaacacccagtttacagccgtgggcaaggagttcaatcacctggagaagcgcatcgagaacctgaataagaaggtggacgatggctttctggacatctggacctacaacgccgagctgctggtgctgctggagaatgagaggacactggactaccacgattccaacgtgaagaatctgtatgagaaggtgcgctctcagctgaagaacaatgccaaggagatcggcaacggctgcttcgagttttaccacaagtgcgacaacacctgtatggagtctgtgaagaatggcacatacgattatcccaagtatagcgaggaggccaagctgaatcgggaggagatcgatggcgtgaagctggagagcaccagaatctaccagatcctggccatctattccacagtggcctctagcctggtgctggtggtgagcctgggagcaatctccttctggatgtgctctaacggcagcctgcagtgcaggatctgtatc

SEQ ID NO: 106 - DNA, 1689 bp, synthetic construct
  misc_feature 1..1689: note = synthetically-generated coding sequence
  source 1..1689: mol_type = other DNA
atgaaggtgaagctgctggtgctgctgtgcaccttcacagccacctacgccgacacaatctgtatcggctatcacgccaacaatagcacagacaccgtggataccatcctggagaagaacgtgacagtgacccactctgtgaatctgctggagaacagccacaatggcaagctgtgcctgctgaagggcatcgccccactgcagctgggaaactgctccgtggcaggatggatcctgggaaatccagagtgtgagctgctgatctctaaggagtcttggagctacatcgtggagaagccaaaccccgagaatggcacatgctaccccggcgacttcatcaactatgaggagctgagggagcagctgagctccgtgtctagcctggagcggttcgagatctttcctaaggagtcctcttggccaaatcacacagtgaccggcgtgtccgcctcttgtagccacaacggcgagagctccttttaccggaatctgctgtggctgaccggcaagaacggcctgtaccctaatctgtccaagtcttatgccaacaataaggagaaggaggtgctggtgctgtggggagtgcaccacccacctaacatcggcgatcagagagccctgtaccacacagagaatgcctacgtgagcgtggtgtctagccactactctaggaagttcacccccgagatcgccaagaggcctaaggtgcgcgaccaggagggacgcatcaactactattggacactgctggagcccggcgataccatcatctttgaggccaacggcaatctgatcgcccctagatatgccttcgccctgagcaggggatttggatccggcatcatcaactctaatgcccctatggacaagtgcgatgccaagtgtcagaccccacagggcgccatcaactcctctctgccattccagaatgtgcaccccgtgacaatcggcgagtgtcctaagtacgtgcggagcgccaagctgagaatggtgaccggcctgcggaacatcccaagcatccagtccagaggactgctgggagcaatcgcaggctttatcgagggaggctggacaggcatgatcgacggctggtacggctatcaccaccagaacgcacagggaagcggatatgcagcagaccagaagtccacacagaatgccatcgatgagatcaccaacaaggtcaattccgtgatcgagaagatgaacatccagttcaccgccgtgggcaaggagtttaataagctggagcggagaatggagaacctgaataagaaggtggacgatggcttcatcgatatctggacatacaacgccgagctgctgatcctgctggagaatgagcggaccctggactttcacgatagcaacgtgaagaatctgtatgagaaggtgagaaaccagctgaagaacaatgccaaggaagtgggcaatggctgcttcgagttttaccacaagtgcaacgacgagtgtatggagtccgtgaagaatggcatctacgattatcccaagtattctgaggagagcaagctgaacagggagaagatcgatggcgtgaagctggagtctatgggcgtgtaccagatcctggccatctatagcaccgtggcaagctccctggtgctgctggtgagcctgggagccatctccttttggatgtgctccggccactcttgcagaatctgtatc

SEQ ID NO: 107 - DNA, 1698 bp, synthetic construct
  misc_feature 1..1698: note = synthetically-generated coding sequence
  source 1..1698: mol_type = other DNA
atggaggccatcctggtggtgctgctgtacacctttaccacagccaacgccgacacactgtgcgtgggctatcacgccaacaatagcaccgacacagtggataccgtgctggagcggaatgtgaccgtgacacactccgtgaacctgctggaggattctcacaatggcaagctgtgcagactgaagggcatcgcccctctgcagctgggcaagtgcaacatcgccggctggctgctgggcaatccagagtgtgagtccctgttttctaaggagagctggtcctacatcgtggagacccccaaccctgagaatggcacatgctaccctggccacttcgccgactatgaggagctgagggagcagctgaacagcgtgagcagcttcgagcggttcgagatgttcccaaagacctctagctggcccgaccacgattccaataagggagtgaccacagcatgtccacacgcaggagcaaagggcttttacaagaacctgatctggctgacaaagaagggcaatagctaccccaagctgtctcagagctatatcaacgataagggcaaggagatcctggtgctgtggggcatccaccacccaagcaccacagccgaccagcagtccctgtaccagaatgccgatacctacgtgttcgtgggcacaagcaagtactccaagaagttcaagcctgagatcgccacccggccaaaggtgagagaccaggagcggagaatgaactactattggaccctgatcgagccaggcgataagatcacatttgaggccaacggcaatctggtggtgccccggtatgccttcaccatggagagaaacgccggctccggcatcatcatctctgacacaagcgtgcacgattgcaataccacatgtcagacccccgagggcgccatcaacacatccctgcccttccacaatatccaccctatcaccatcggcgagtgccccaagtacgtgaggtctaccaagctgcgcatggtgacaggcctgaggaacgtgccttccgtgcagtctaggggactgtttggagcaatcgcaggcttcatcgagggaggatggaccggaatgatggacggatggtacggctatcaccaccagaatggccagggctctggctatgccgccgatcagaagagcacccagaacgccatcaatggcatcacaaacaaggtcaattccgtgatcgacaagatgaacacccagtttacagccgtgggcaaggagttcaataagctggagaagaggatggagaacctgaataagaaggtggacgatggctttatcgacgtgtggacctacaacgccgagctgctgatcctgctggagaatgagcgcacactggactaccacgattccaaggtgaagaacctgtatgagaaggtgaagtctcagctgaagaacaatgccaaggagaccggcaatggctgcttcgagttttaccacaagtgcaacaatgagtgtatggagtctgtgaagaacggcacatacgactatcctcggtatagcgaggaggccaagctgaatagagagaagatcgatggcgtgaagctggagagcacccgggtgtaccagatcctggccatctattccacagccgcctcctctctggtgctggtggtgtctctgggcgagatcagcttctggatgtgcagcaacggctccctgaggtgccgcatctgtatc

SEQ ID NO: 108 - DNA, 1692 bp, synthetic construct
  misc_feature 1..1692: note = synthetically-generated coding sequence
  source 1..1692: mol_type = other DNA
atgaagaccatcatcgccctgtcttatatcctgtgcctggtgttcgcccagaagctgccaggcaatgacaacaatagcaccgccacactgtgcctgggacaccacgccgtgcccaacggcacaatcgtgaagaccatcacaaatgatcagatcgaggtgaccaacgccacagagctggtgcagagctccaccggcgagatctgcgacagccctcaccagatcctggatggcgagaactgtacactgatcgacgcactgctgggcgacccacagtgcgatggcttccagaataagaagtgggatctgtttgtggagcggtctaaggcctacagcaactgttacccctatgacgtgcctgattatgcctccctgagatctctggtggcctctagcggcaccctggagttcaacaatgagtcttttaattggaccggcgtgacacagaacggcacatcctctgcctgcatccggagatctaatagcttctttagcaggctgaattggctgactcacctgaacttcaagtaccccgccctgaacgtgacaatgcctaacaatgagcagtttgacaagctgtatatctggggagtgcaccacccaggcaccgacaaggatcagatcttcctgtacgcacagtccggaaggatcaccgtgtccacaaagagatctcagcaggccgtgatccctaatatcggatctaggccaaggaggatcccaagccgcatctccatctattggaccatcgtgaagcctggcgacatcctgctgatcaacagcacaggcaatctgatcgccccaaggggctacttcaagatccgctctggcaagagctccatcatgcggagcgacgccccaatcggcaagtgctccgagtgtatcacccccaatggctctatccctaacgataagccatttcagaacgtgaatcggatcacatacggcgcctgtcccagatatgtgaagcagaccctgaagctggccacaggcatgaggaacgtgcctgagaagcagaccaggggaatcttcggagcaatcgcaggctttatcgagaatggctgggagggcatggtggacggctggtacggctttcggcaccagaacagcgagggaagaggacaggcagcagacctgaagtccacccaggcagccatcgatcagatcaacggcaagctgaataggctgatcggcaagacaaatgagaagttccaccagatcgagaaggagttttccgaggtggagggccgcatccaggatctggagaagtacgtggaggacaccaagatcgatctgtggagctataatgccgagctgctggtggccctggagaaccagcacaccatcgacctgacagattccgagatgaacaagctgttcgagaagaccaagaagcagctgcgggagaatgccgaggacatgggcaacggctgctttaagatctatcacaagtgcgataatgcctgtatcggctccatcagaaacggcacatacgaccacgacgtgtacagggacgaggccctgaacaatcgcttccagatcaagggcgtggagctgaagtctggctacaaggattggatcctgtggatcagcttcgccatctcctgctttctgctgtgcgtggccctgctgggctttatcatgtgggcctgccagaagggcaacatccggtgtaatatcagatgcaacatctgtatc

SEQ ID NO: 109 - DNA, 1698 bp, synthetic construct
  misc_feature 1..1698: note = synthetically-generated coding sequence
  source 1..1698: mol_type = other DNA
atgaagaccatcatcgccctgtctcacatcctgtgcctggtgttcgcccagaagatcccaggcaacgacaatagcaccgccacactgtgcatcggacaccacgccgtgcccaacggcatgatcgtgaagaccatcacaaatgatagaatcgaggtgaccaacgccacagagctggtgcagaatagctccatcggcgagatctgcgacagcccccaccagatcctggatggcgagaattgtacactgatcgacgcactgctgggcgaccctcactgcgatggctttcagaacgagaagtgggatctgttcgtggagagatctaaggcctttagcaattgttacccctatgacgtgcctgattacgcctccctgaggtctctggtggcctctagcggcaccctggagttcaagaatgagtcctttaactggaccggcgtggcccagaacggcacatcctctgcctgcatccggagaagctcctctagcttcttttctaggctgaattggctgacccacctgaactacacatatccagccctgaatgtgacaatgcccaacaaggagcagttcgacaagctgtacatctggggagtgcaccacccaggcaccgacaaggatcagatctttctgtatgcccagtcctctggccgcatcaccgtgtccacaaagcggtctcagcagacagccatcccaaatatcggaagcaggccaaggatcagggacatccctagccgcatctccatctactggaccatcgtgaagcccggcgacgtgctggtcatcaactccaatggcaacctgatcgcccctcgcggctatttcaagatccagtccggcaagagctccatcatgcggtctgacgcccccatcggcaagtgcaagagcgagtgtatcacacctaatggctctatcagcaacgataagccatttcagaatgtgaacaagatcacctacggcgcctgtcctagatatgtgaagcactccaccctgaagctggccacaggcatgagaaacgtgccagagaagcagaccaggggactgttcggagcaatcgcaggctttatcgagaacggctgggagggcatgaaggacggctggtacggcttcagacaccagaatagcgagggaaggggacaggcagcagatctgaagtccacacaggccgccatcaatcagatcaacggcaagctgaaccgcctgatcggcaagaccaatgagaagttccaccagatcgagaaggagtttagcgaggtggagggaagggtgcaggacctggagaagtacgtggaggactctaagatcgatctgtggagctataacgccggcctgctggtggccctggagaatcagcacaccatcgacctgacagattccgagatgaacaagctgttcgagagaaccaggaagcagctgagagagaatgccgaggacatgggcaacggctgttttacaatctaccacaagtgcgataacgcctgtatcggctctatcaggaatggcacctacgaccacaacgtgtatcgcgatgaggccctgaataagcggttccagatcaagggcatcgagctgaagtccggctataaggattggatcctgtggatcagcttcgccatctcctgctttctgctgtgcgtggccctgctgggctttatcatgtgggcctgccagaagggcaatatccggtgcaacatctgtatc

SEQ ID NO: 110 - DNA, 1698 bp, synthetic construct
  misc_feature 1..1698: note = synthetically-generated coding sequence
  source 1..1698: mol_type = other DNA
atgaagaccatcatcgccctgtcttatatcctgtgcctggtgttcgcccagaagctgcctggcaacgacaatagcaccgccacactgtgcctgggacaccacgccgtgccaaatggcacaatcgtgaagaccatcacaaacgatcagatcgaggtgaccaatgccacagagctggtgcagaacagctccatcggcgagatctgcgactccccacaccagatcctggatggcgagaactgtaccctgatcgacgcactgctgggcgacccacagtgcgatggcttccagaataagaagtgggatctgtttgtggagagatctaaggcctacagcaactgttacccctatgacgtgcctgattatgcctccctgaggtctctggtggcctctagcggcaccctggagttcaacaatgagagctttaattggaccggcgtgacacagaacggcacatcctctgcctgcatccggagaagcaacaattccttcttttctagactgaactggctgactcacctgaatttcaagtaccctgccctgaatgtgacaatgccaaacaatgagcagtttgacaagctgtatatctggggagtgcaccaccctggcaccgacaaggatcagatcttcctgtacgcacagagctccggaaggatcaccgtgtccacaaagcggtctcagcaggccgtgatccctaacatcggaagcaggccaaggatcagggacatcccaagccgcatctccatctattggaccatcgtgaagccaggcgatatcctgctgatcaactccacaggcaatctgatcgcccccagaggctacttcaagatcaggtctggcaagtctagcatcatgcggagcgacgcccccatcggcaagtgcaagtccgagtgtatcacccctaacggctctatcccaaatgataagccctttcagaacgtgaatagaatcacatacggcgcctgtcccagatatgtgaagcagaataccctgaagctggccacaggcatgcgcaacgtgcctgagaagcagaccaggggaatcttcggagcaatcgcaggctttatcgagaatggctgggagggcatggtggacggctggtacggctttagacaccagaacagcgagggaaggggacaggcagcagacctgaagtccacccaggccgccatcgatcagatcaacggcaagctgaatcgcctgatcggcaagacaaacgagaagttccaccagatcgagaaggagttttccgaggtggagggccggatccaggatctggagaagtacgtggaggacaccaagatcgatctgtggtcctataatgccgagctgctggtggccctggagaaccagcacaccatcgacctgacagattctgagatgaacaagctgttcgagaagaccaagaagcagctgagagagaacgccgaggacatgggcaatggctgttttaagatctatcacaagtgcgataatgcctgtatcggctctatcaggaacggcacatacgaccacgacgtgtaccgcgacgaggccctgaacaatcggttccagatcaagggcgtggagctgaagagcggctacaaggattggatcctgtggatcagcttcgccatctcctgctttctgctgtgcgtggccctgctgggctttatcatgtgggcctgccagaagggcaacatcaggtgcaatatctgtatc

SEQ ID NO: 111 - DNA, 1698 bp, synthetic construct
  misc_feature 1..1698: note = synthetically-generated coding sequence
  source 1..1698: mol_type = other DNA
atgaagaccatcatcgccctgtcccacatcctgtgcctggtgttcgcccagaagatccccggcaacgacaattccaccgcaatgctgtgcctgggacaccacgccgtgtctaatggcacaatcgtgaagaccatcacaaatgatcgcatcgaggtgaccaacgccacagagctggtgcagagctcctctaccggcgagatctgcgacagccctcaccggatcctggatggcaagaactgtacactgatcgacgcactgctgggcgacccacactgcgatggcttccagaataaggagtgggatctgtttgtggagcggagcaaggcccactctaactgttacccctatgacgtgcctgattacgtgagcctgcggtccctggtggcaagctccggcaccctggagttcaagaatgagtcttttaactggaccggcgtggcccagaacggcacatctagcgcctgcatccggagatcctctagctccttctttagcagactgaattggctgacccacctgaactacacatatccagccctgaatgtgacaatgcccaacaatgagaagttcgacaagctgtacatctggggagtgcaccacccaggcaccgacaacgatcagatctttctgtatgcacaggccagcggaaggatcaccgtgagcacaaagcggtcccagcagacagtgatcccaaatatcggatccaggccacgcgtgcggaacatcccttctaggatcagcatctactggaccatcgtgaagcccggcgacgtgctggtcatcaacagcaatggcaacctgatcgcccctcgcggctatttcaagatccagagcggcaagtctagcatcatgcggtccgacgcccctatcggcaagtgcaattccgagtgtatcacacctaatggctccatctctaacgataagccatttcagaatgtgaacaagatcacctacggcgcctgtccaagatatgtgaagcactccaccctgaagctggccacaggcatgaggaacgtgcccgagagacagacaaggggcatcttcggcgccatcgccgtgtttatcgagaatggctgggagggcatgatggacggctggtacggcttccgccaccagaactctgagggcaccggacaggcagcagatctgaagagcacacaggccgccatcaatcagatcaacggcaagctgaatagactgatcgagaagaccaacgagaagttccaccagatcgagaaggagttttctgaggtggagggcagggtgcaggacctggagaagtacgtggaggactccaagatcgatctgtggtcttataatgcaggactgctggtggccctggagaaccagcacaccatccacctgacagatagcgagatgaacaagctgttcgagagaaccaagaagcagctgagggagaatgccgaggacatgggcaacggctgttttacaatctaccacaagtgcgataatgcctgtatcgagtccatcagaaatggcacctacgaccacaacgtgtatagagatgaggccctgaacaagaggttccagatcaagggcatcgagctgaagtctggctataaggactgggtgctgtggatctctttcgccatcagctgctttctgctgtgcgtggtgctgctgggctttatcatgtgggcctgccagcgcggcaatatccggtgcaacatctgtatc

SEQ ID NO: 112 - DNA, 1698 bp, synthetic construct
  misc_feature 1..1698: note = synthetically-generated coding sequence
  source 1..1698: mol_type = other DNA
atgagaaccatcatcgccctgagctatatcttctgtctggtgtttgcccagaagctgccagagaacgacaattccaccgccacactgtgcatcggacaccacgccgtgcccaacggcacactggtgaagaccatcacaaacgatcaggtggaggtgaccaatgccacagagctggtgcagagctcctctaccggaggaatctgcgactccccacaccagatcctggatggcaagaattgtacactggtggacgcactgctgggcgaccctcactgcgatggcttccagaacgagaagtgggatctgttcgtggagagatctaaggcctttagcaattgttacccatatgacgtgcaggattacgcctctctgaggagcctgatcgcaagctccggcaccctggagttcaacaatgagagctttaactgggccggcgtgacccagaatggcacatctagcgcctgcaagcggagatctaactcctctttctttagcaggctgaattggctgacccacctgaagttcaagtacccagccctgaacgtgacaatgcccaataaggagcagtttgacaagctgtatatctggggagtgcaccacccatccaccgactctgatcagatctccctgtacgcccaggcctctggcagagtgaccgtgtccacaaagaggtctcagcagacagccatcccaaacatcggctccaggccccgcatccggaatatccctagccgcgtgtccatctattggaccatcgtgaagcccggcgatatcctgctgatcaactgtacaggcaatctgatcgcccctcgcggctacttcaagatccggaacggcaagagctccatcatgcggtccaacgcccctatcggcaagtgcaatagcgcctgtatcaccccaaacggctccatccccaatggcaagccttttcagaacgtgaatagagtgacatacggcgcctgccctagatatgtgaagcagtctaccctgaagctggccacaggcatgcgcaacgtgccagagaagcagaccaggggactgttcggagcaatcgcaggctttatcgagaacggctgggagggcatgaaggacggctggtacggcttccggcaccagaattccgagggaatcggacaggcagcagacctgaagtctacacaggccgccgtggatcagatcaacggcaagctgaatcgcgtgatcgagaagaccaacgagaagttccaccagatcgagaaggagtttacagaggtggagggccggatccaggacatcgagaagtacgtggaggacaccaaggtggatctgtggtcttataacgccgagctgctggtgagcctggagaatcagcacaccatcgacatgacagatagcgagatgaataagctgttcgagagaaccaggaagcagctgagagagaacgccgaggatatcggcaatggctgttttaagatctatcacaagtgcaacaatgcctgtatcggctctatcaggaacgagacatacgaccacaacgtgtaccgcgatgaggccctgaacaatcggttccacatcaagggcgtggagctgaagagcggctacaagaactggatcctgtggatcagcttcgccacctcctgctttctgctgtgcatcgtgctgctgggctttatcatgtgggcctgccagaagggcaacatcaagtgcaatatctgtatc

SEQ ID NO: 113 - DNA, 1713 bp, synthetic construct
  misc_feature 1..1713: note = synthetically-generated coding sequence
  source 1..1713: mol_type = other DNA
atgaagaccatcatcgccttctcttgcatcctgtgcctgatctttgcccagaagctgcccggctccgacaacaattctatggccaccctgtgcctgggacaccacgcagtgcctaatggcacactggtgaagaccatcacagacgatcagatcgaggtgaccaacgccacagagctggtgcagagctcctctaccggcaggatctgtaattcccctggccaccagatcctggatggcaagaactgcacactgatcgacgccctgctgggcgatccacactgtgacgatttccagaataagtgggacctgtttgtggagcggagcaccgcctactccggcaactgctatccctactatgtgcctgattacgccagcctgagagagcagctgtccctggtggccagctccggcaccctggagttcacacaggagtcttttaattggaccggagtggcacaggacggctctagctacgcctgtcggagaggcagcgtgaacaattctttctttagccgcctgaactggctgtatctgaattacaagtatcccgccctgaacgtgacaatgcctaacaatgacaagttcgataagctgtacatctggggagtgcaccacccaggaaccgacaaggatcagacaaatctgtatgtgcaggccagcggcagggtggtgtctaccaagcgcagccagcagacagtgatccctaacatcggctcccggccatgggtgagaggcgtgtcctctatcatctctatctactggaccatcgtgaagcctggcgacatcctgctgatcaacagcacaggcaatctgatcgccccaaggggctatttcaagatccagtccggcaagagctccggcatcatgcgctctgacgccccaatcgattgcaacagcgagtgtatcacccccaacggctccatcccaaatgataagccctttcagaacgtgaataggatcacatacggcgcctgcccacgctatgtgaagcagaataccctgaagctggccacaggcatgcggaacgtgcccgagaagcagaccagaggcatcttcggcgccatcgccggctttatcgagaatggctgggagggcatggtggacggctggtacggcttccggcaccagaactctgagggaaccggacaggcagcagatctgaagagcacccaggcagccatcaaccagatcacaggcaagctgaatagagtgatcaagaagaccaacgagaagttccaccagatcgagaaggagtttagcgaggtggagggaaggatccaggacctggagaagtacgtggaggacaccaagatcgatctgtggtcctataatgccgagctgctggtggccctggagaaccagcacaccatcgacctgacagattctgagatgaacaagctgttcgagaggaccaggaagcagctgagggagaacgcagaggacatgggcaatggctgctttaagatctaccacaagtgcgataatgcctgtatcggctccatcagaaacggcacatacgaccacgacgtgtaccgggacgaggccctgaacaatagattccagatcaagggcgtgcagctgaagagcggctataaggattggatcctgtggatctccttcgccatctcttgctttctgctgtgcgtggtgctgctgggctttatctccatgtgggcctgtcagaagggcaacatcagatgcaatatctgtatc

SEQ ID NO: 114 - DNA, 1698 bp, synthetic construct
  misc_feature 1..1698: note = synthetically-generated coding sequence
  source 1..1698: mol_type = other DNA
atgaagaccatcatcgccttcagctgcatcctgtgcctgatctttgcccagaagctgcctggctccgacaattctaccgccaccctgtgcctgggacaccacgcagtgccaaacggcacaatggtgaagaccatcacagacgatcaggtggaggtgaccaatgccacagagctggtgcagagctcctctaccggccggatctgcaatagcccacaccagatcctggatggcaagaactgtacactgatcgactccctgctgggcgatccccactgcgacgatttccagaataaggagtgggacctgtttgtggagaggtctaaggcctacagcaactgttatccctactatgtgcctgattacgccaccctgcgctccctggtggccagctccggcaatctggagttcacccaggagtcttttaactggacaggagtggcacaggacggctctagctacgcatgccggagaggcagcgtgaactccttcttttctagactgaattggctgtataacctgaattacaagtatcctgagcagaacgtgaccatgccaaacaatgacaagttcgataagctgtacatctggggagtgcaccaccctggaaccgacaaggatcagacaaatctgtatgtgcaggccagcggcagagtgatcgtgagcaccaagcggagccagcagacaatcatcccaaacatcggctctcggccctgggtgagaggcgtgtcctctatcatcagcatccactggaccatcgtgaagccaggcgacatcctgctgatcaactccacaggcaatctgatcgcccccagaggctacttcaagatccagaatggcaagagctccatcatgagatccgacgcccacatcgatgagtgcaactctgagtgtatcacccccaacggctctatcagcaatgataagccttttcagaacgtgaataagatcacatacggcgcctgccccaggtatatcaagcagaataccctgaagctggccacaggcatgaggaacatccctgagaagcagacccgcggcatcttcggagcaatcgcaggctttatcgagaacggctgggagggcatggtgaatggctggtatggcttccgccaccagaacagcgagggaaccggacaggcagcagacctgaagtccacccaggccgccatcaaccagatcacaggcaagctgaatagagtgatcaagaagaccaacgagaagttccaccagatcgagaaggagttttctgaggtggagggcagaatccaggatctggagaagtacgtggaggacaccaagatcgatatctggtcctataatgccgagctgctggtggccctggagaaccagcacaccatcgacctgacagatagcgagatgtccaagctgttcgagcggaccaggcgccagctgagagagaacgccgaggacatcggcaatggctgttttaagatctaccacaagtgcgataatagctgtatggagtccatcaggaacggcacatacgaccacgatatctatcggaacgaggccctgaacaatagattccagatcaagggcgtgcagctgaagagcggctataaggactggatcctgtggatctctttcgccatcagctgctttctgctgtgcgtggtgctgctgggctttatcatgtgggcctgccagaggggcaacatccgctgcaatatctgcgtg

SEQ ID NO: 115 - DNA, 1698 bp, synthetic construct
  misc_feature 1..1698: note = synthetically-generated coding sequence
  source 1..1698: mol_type = other DNA
atgaaggccatcctggtggtgctgctgtacacctttaccacagccaacgccgacacactgtgcatcggctatcacgccaacaatagcaccgacacagtggataccgtgctggagaagaatgtgaccgtgacacacagcgtgaacctgctggaggattcccacaatggcaagctgtgcaagctgaggggagtggcaccactgcacctgggcaagtgcaacatcgcaggatggctgctgggaaatccagagtgtgagagcctgtccaccgccagctcctggtcctacatcgtggagacctctaacagcgacaatggcacatgctacccaggcgacttcatcaactatgaggagctgagggagcagctgagcagcgtgagcagcttcgagcggttcgagatcttccccaagaccagctcctggcctaaccacgacaccaataggggagtgacagcagcatgtccacacgcaggaacaaactccttctaccgcaatctgatctggctggtgaagaagggcaattcttaccctaagctgtccaagtcttatatcaacaataaggagaaggaggtgctggtgctgtgggcaatccaccaccccagcacctccgccgaccagcagagcctgtaccagaacgccgatgcctacgtgttcgtgggctctagcaggtactcccgcaagttcgagccagagatcgcaaccaggccaaaggtgagagaccaggccggcaggatgaattactattggacactggtggagcccggcgataagatcacctttgaggccacaggcaacctggtggtgcctcggtatgccttcgccctgaagagaaattctggcagcggcatcatcatctccgatacctctgtgcacgactgcgataccacatgtcagacccctaacggcgccatcaatacaagcctgcctttccagaacatccacccagtgacaatcggcgagtgccctaagtacgtgaagtccaccaagctgaggatggccacaggcctgcgcaatatcccaagcatccagtcccgcggcctgtttggagcaatcgcaggcttcatcgagggaggatggaccggaatgatcgacggatggtacggctatcaccaccagaacgagcagggctctggctatgccgccgacctgaagagcacccagaatgccatcgatggcatcacaaacaaggtcaatagcgtgatcgagaagatgaacacccagtttacagccgtgggcaaggagttcaataagctggagcggagaatggagaacctgaataagaaggtggacgatggctttctggatatctggacctacaacgccgagctgctggtgctgctggagaatgagcggacactggactaccacgattccaacgtgaagaatctgtatgagaaggtgagatctcagctgaagaacaatgccaaggagatcggcaacggctgcttcgagttttaccacaagtgcaacaatgagtgtatggagtctgtgaagaacggcacctacgactatcccaagtatagcgaggaggccaagctgaatcgggaggagatcgatggcgtgaagctggagagcaccagaatctaccagatcctggccatctattccacagtggcctcctctctggtgctgctggtgtccctgggcgccatctctttctggatgtgctctaacggcagcctgcagtgccggatctgtatc

SEQ ID NO: 116 - DNA, 1695 bp, synthetic construct
  misc_feature 1..1695: note = synthetically-generated coding sequence
  source 1..1695: mol_type = other DNA
atgaaggtgaagctgctgatcctgctgtgcacctttacagccacctacgccgacacaatctgtatcggctatcacgccaacaattccacagacaccgtggataccatcctggagaagaacgtgacagtgacccactctgtgaatctgctggagaacaggcacaatggcaagctgtgcctgctgaagggaatcgcaccactgcagctgggaaactgcagcgtggcaggatggatcctgggcaatcctgagtgtgagtctctgatcagcaagaagtcctggtcttacatcgtggagacacccaaccctgagaatggcgcctgctaccccggcgagtttgccgattatgaggagctgagggagcagctgagcaccgtgagcagcttcgagcggttcgagatcttcccaaaggagtctagctggcccaaccacacagtgaccggcgtgagcgcctcctgttctcacaacggcgagaggtccttctaccgcaatctgatctggctgaccgtgaagaacggcctgtaccctaatctgagcaagtcctatgagaatgacaagggcaaggaggtgctgatcctgtggggcgtgcaccacccatccaacatcggcgatcagcgcacactgtaccacaccgagaatgcctacgtgagcgtggtgtcctctcactacagccggagattcacacctgagatcaccaagcggccaaaggtgagagaccaggagggccggatcaactactattggacactgctggagcctggcgataccatcatctttgaggccaacggcaatctgatcgccccatggtatgccttcgccctgagcagaggcctgggatccggcatcatcacatctaatgccccaatggacgagtgcgatgccaagtgtcagaccccacagggagccatcaacagctccctgccctttcagaatgtgcaccctgtgacaatcggcgagtgtccaaagtacgtgaggagcgccaagctgaggatggtgaccggactgaggaacgtgccctccatccagtctagaggcctgctgggagcaatcgcaggcttcatcgagggaggatggacaggaatggtggacggatggtacggctatcaccaccagaatggacagggatccggatatgcagcagatcaggagtctacacagaacgccatcaatggcatcaccaacaaggtcaatagcatcatcgagaagatgaacatccagtttacctccgtgggcaaggagttcaatcacctggagaagaggatcgagaacctgaataagaaggtggacgatggctttctggacgtgtggacatacaacgccgagctgctgatcctgctggagaatgagcgcaccctggacttccacgattccaacgtgaagtctctgtatgagaaggtgaagagccagctgaagaacaatgccaaggaagtgggcaatggctgcttcgagttttaccacaagtgcgacgatacatgtatggagtccgtgaagaacggcacctacaattatcctaagtatagcgaggagtccaagctgaaccgggagaagatcgacggcgtgaagctggattctatgggcgtgtacagaatcctggccatctatagcaccgtggcctctagcctggtgctggtggtgagcctgggagcaatctccttttggatgtgctctaacggcagcctgcagtgccgggtgtgcatc

SEQ ID NO: 117 - DNA, 1698 bp, synthetic construct
  misc_feature 1..1698: note = synthetically-generated coding sequence
  source 1..1698: mol_type = other DNA
atggaggccaagctgttcgtgctgttttgcgccttcaccgccctgaaggccgacacaatctgcgtgggctaccacgccaacaatagcaccgagacagtggataccgtgctggagaagaacgtggccgtgacacactccgtgaacctgctggaggacaagcacaatggcaagctgtgcaagctgggaggaatcgcaccactgcacctgggcaagtgcaacatcgccggctggatcctgggcaatcctgagtgtgagctgctgatcagcaaggagtcttggagctacatcgtggaggccccaaactccgacaatggagcatgctacccaggacagttcgcagattatgaggagctgcgggagcacctgagctccgtgtctagctttgagaagttcgagatctttccaaaggcctcctcttggcccaaccacgattctaataagggagtgaccgcagcatgtccttacgcaggcgccaacagcttttataggaatctgctgtggatcgtgaagaagggcaacagctacccaaagatcaataagtcctacatcaacaataagggcaaggaggtgctggtgctgtggggaatccaccacccacctacctccacagaccagcagtctctgtacaagaacgccgatgcctacgtgttcgtgggcacctcccggtactctaagaagtttaagcctgagatcgccatcaggccaaaggtgcgcgaccaggagggcagaatgaattactattggaccctgctggaccagggcgataccatcacattcgaggcaacaggaaacctggtggcaccaagatatgcctttgccatggagcgcaatgccggcagcggcatcatcatctccgacacccctgtgcacgattgcaacaccacatgtcagacaccaaagggcgccatcaacagcaatctgcccttccagaatgtgcaccctatcaccatcggcgagtgtccaaagtacgtgcggtccaccaagctgagaatggtgacaggcctgcggaacatccccagcgtgcagtccagaggcctgttcggagcaatcgcaggctttctggagggaggatggacaggcatggtgaacggctggtacggctatcaccaccagaatgaccagggctctggctatgccgccgatcagaagagcacccagatcgccatcgacggcatctctaacaaggtcaatagcgtgatcgagaagatgaatatccagttcacagccgtgggcaaggagtttagccacctggagcggagaatcgagaacctgaataagaaggtggacgatggcctgctggacgtgtggacctacaacgccgagatgctggtgctgctggagaatgagaggacactggacttccacgacttcaacgtgaagaatctgtacgagaaggtgaagtcccagctgcgcaacaatgccaaggagatcggcaacggctgcttcgagttttatcacaagtgcgacaacacctgtatggagtccgtgaggaatggcacatacgattatcctaagtactatgaggagtctaagctgaatcgcgaggagatcgatggcgtgaagctggagtccatgggcgtgtaccagatcctggccatctattctaccgcagccagctccctggtgctgctggtgtccctgggagccgtgtctttctggatgtgctctaacggcagcctgcagtgcaagatctgtatc

SEQ ID NO: 118 - DNA, 1713 bp, synthetic construct
  misc_feature 1..1713: note = synthetically-generated coding sequence
  source 1..1713: mol_type = other DNA
atgaagaccatcatcgccttctcctgcatcctgtgcctgatcttcgcccagaagctgcccggcagcgacaacaactccatggccaccctgtgcctgggacaccacgccgtgccaaacggcaccctggtgaagaccatcaccgacgaccagatcgaggtgaccaacgccaccgagctggtgcagtccagctccaccggaaggatctgcaacagcccaggacaccagatcctggacggcaagaactgcaccctgatcgacgctctgctgggcgacccacactgcgacgacttccagaacaagtgggacctgttcgtggagcgcagcaccgcctactccggcaactgctacccctactacgtgccagactacgccagcctgagggagcagctgtccctggtggctagctccggcaccctggagttcacccaggagtccttcaactggaccggcgtggcccaggacggaagctcctacgcttgcaggaggggaagcgtgaacaacagcttcttctccagactgaactggctgtacctgaactacaagtaccccgccctgaacgtgaccatgccaaacaacgacaagttcgacaagctgtacatctggggagtgcaccacccaggcaccgacaaggaccagaccaacctgtacgtgcaggcctccggaagggtggtgagcaccaagagatcccagcagaccgtgatccccaacatcggatccaggccatgggtgcggggcgtgagctccatcatcagcatctactggaccatcgtgaagcccggcgacatcctgctgatcaactccaccggcaacctgatcgccccaaggggctacttcaagatccagagcggcaagagctccggcatcatgagaagcgacgcccccatcgactgcaactccgagtgcatcaccccaaacggcagcatccccaacgacaagccattccagaacgtgaacaggatcacctacggcgcctgccccagatacgtgaagcagaacaccctgaagctggccaccggcatgcgcaacgtgccagagaagcagaccaggggaatcttcggagctatcgctggcttcatcgagaacggctgggagggcatggtggacggctggtacggcttccgccaccagaactccgagggcaccggacaggctgctgacctgaagagcacccaggccgccatcaaccagatcaccggcaagctgaaccgcgtgatcaagaagaccaacgagaagttccaccagatcgagaaggagttctccgaggtggagggcagaatccaggacctggagaagtacgtggaggacaccaagatcgacctgtggtcctacaacgccgagctgctggtggccctggagaaccagcacaccatcgacctgaccgacagcgagatgaacaagctgttcgagaggaccagaaagcagctgcgcgagaacgccgaggacatgggcaacggctgcttcaagatctaccacaagtgcgacaacgcctgcatcggcagcatccggaacggcacctacgaccacgacgtgtaccgcgacgaggccctgaacaaccggttccagatcaagggcgtgcagctgaagtccggctacaaggactggatcctgtggatcagcttcgccatctcctgcttcctgctgtgcgtggtgctgctgggcttcatcagcatgtgggcctgccagaagggcaacatccggtgcaacatctgcatc

SEQ ID NO: 119 - DNA, 1698 bp, synthetic construct
  misc_feature 1..1698: note = synthetically-generated coding sequence
  source 1..1698: mol_type = other DNA
atgaagaccatcatcgccttctcctgcatcctgtgcctgatcttcgcccagaagctgccaggaagcgacaactccaccgccaccctgtgcctgggacaccacgccgtgccaaacggcaccatggtgaagaccatcaccgacgaccaggtggaggtgaccaacgccaccgagctggtgcagtccagctccaccggaaggatctgcaactccccacaccagatcctggacggcaagaactgcaccctgatcgacagcctgctgggcgacccacactgcgacgacttccagaacaaggagtgggacctgttcgtggagaggtccaaggcctacagcaactgctacccctactacgtgccagactacgccaccctgagatccctggtggccagctccggcaacctggagttcacccaggagagcttcaactggaccggcgtggcccaggacggaagctcctacgcttgcaggaggggcagcgtgaactccttcttcagccggctgaactggctgtacaacctgaactacaagtaccccgagcagaacgtgaccatgccaaacaacgacaagttcgacaagctgtacatctggggagtgcaccacccaggcaccgacaaggaccagaccaacctgtacgtgcaggcctccggacgcgtgatcgtgtccaccaagagaagccagcagaccatcatccccaacatcggatccaggccatgggtgcggggcgtgagctccatcatcagcatccactggaccatcgtgaagcccggcgacatcctgctgatcaacagcaccggaaacctgatcgctccaaggggctacttcaagatccagaacggcaagagctccatcatgcggtccgacgcccacatcgacgagtgcaacagcgagtgcatcacccccaacggcagcatctccaacgacaagccattccagaacgtgaacaagatcacctacggcgcctgccccaggtacatcaagcagaacaccctgaagctggccaccggcatgaggaacatcccagagaagcagaccagaggcatcttcggcgccatcgccggcttcatcgagaacggctgggagggcatggtgaacggctggtacggcttcagacaccagaactccgagggcaccggacaggctgctgacctgaagagcacccaggccgccatcaaccagatcaccggcaagctgaaccgcgtgatcaagaagaccaacgagaagttccaccagatcgagaaggagttctccgaggtggagggaaggatccaggacctggagaagtacgtggaggacaccaagatcgacatctggagctacaacgccgagctgctggtggccctggagaaccagcacaccatcgacctgaccgactccgagatgagcaagctgttcgagcgcaccaggagacagctgcgggagaacgccgaggacatcggcaacggctgcttcaagatctaccacaagtgcgacaactcctgcatggagagcatcaggaacggcacctacgaccacgacatctaccgcaacgaggccctgaacaaccggttccagatcaagggcgtgcagctgaagagcggctacaaggactggatcctgtggatctccttcgccatcagctgcttcctgctgtgcgtggtgctgctgggcttcatcatgtgggcctgccagaggggcaacatcagatgcaacatctgcgtg

SEQ ID NO: 120 - DNA, 1698 bp, synthetic construct
  misc_feature 1..1698: note = synthetically-generated coding sequence
  source 1..1698: mol_type = other DNA
atgaagaccatcatcgccttctcctgcatcctgtgcctgatcttcgcccagaagctgcccggcagcgacaactccatggccaccctgtgcctgggacaccacgccgtgccaaacggcaccctggtgaagaccatcaccgacgaccagatcgaggtgaccaacgccaccgagctggtgcagtccagctccaccggcaggatctgcaacagcccccaccagatcctggacggcaagaactgcaccctgatcgacgctctgctgggcgacccacactgcgacgacttccagaacaaggagtgggacctgttcgtggagcgcagcaccgcctacagcaactgctacccctactacgtgccagactacgccagcctgcggtccctggtggctagctccggcaccctggagttcacccaggagtccttcaactggaccggcgtggcccaggacggaagctcctacgcttgcaggaggggcagcgtgaactccttcttcagcagactgaactggctgtacaacctgaactacaagtaccccgagcagaacgtgaccatgccaaacaacgacaagttcgacaagctgtacatctggggagtgcaccacccaggcaccgacaaggaccagaccaacctgtacgtgcaggcctccggacgcgtgatcgtgtccaccaagagaagccagcagaccgtgatccccaacatcggatccaggccatgggtgcggggcgtgagctccatcatcagcatctactggaccatcgtgaagcccggcgacatcctgctgatcaacagcaccggcaacctgatcgccccaaggggctacttcaagatccagtccggcaagagctccatcatgagaagcgacgcccacatcgacgagtgcaactccgagtgcatcacccccaacggcagcatccccaacgacaagccattccagaacgtgaacaggatcacctacggcgcctgccccagatacgtgaagcagaacaccctgaagctggccaccggcatgcgcaacgtgccagagaagcagaccaggggaatcttcggagctatcgctggcttcatcgagaacggctgggagggcatggtggacggctggtacggcttccgccaccagaactccgagggcaccggacaggctgctgacctgaagagcacccaggccgccatcaaccagatcaccggcaagctgaaccgcgtgatcaagaagaccaacgagaagttccaccagatcgagaaggagttcagcgaggtggagggcagaatccaggacctggagaagtacgtggaggacaccaagatcgacctgtggtcctacaacgccgagctgctggtggccctggagaaccagcacaccatcgacctgaccgacagcgagatgaacaagctgttcgagaggaccagaaagcagctgcgcgagaacgccgaggacatgggcaacggctgcttcaagatctaccacaagtgcgacaacgcctgcatcggctccatccggaacggcacctacgaccacgacgtgtaccgcgacgaggccctgaacaaccggttccagatcaagggcgtgcagctgaagagcggctacaaggactggatcctgtggatctccttcgccatcagctgcttcctgctgtgcgtggtgctgctgggcttcatcatgtgggcctgccagaagggcaacatccggtgcaacatctgcatc

SEQ ID NO: 121 - DNA, 1698 bp, synthetic construct
  misc_feature 1..1698: note = synthetically-generated coding sequence
  source 1..1698: mol_type = other DNA
atgaagaccatcatcgccctgtcctacatcctgtgcctggtgttcgcccagaagctgccaggaaacgacaacaacatggccaccctgtgcctgggacaccacgccgtgcccaacggcaccatcgtgaagaccatcaccaacgaccagatcgaggtgaccaacgccaccgagctggtgcagtccaccagcaagggcgagatctgctccagcccacaccagatcctggacggcgagaactgcaccctgatcgacgctctgctgggcgacccacactgcgacgacttccagaacaagaagtgggacctgttcgtggagagatccaaggcccacagcaactgctacccctactacgtgccagactacgccaccctgcgctccctggtggcttccagcggcaacctggagttcacccaggagagcttcaactggaccggagtgacccaggacggagcttccagcgcctgcaagcgccggtccagcaagtccttcttcagccgcctgaactggctgcacaacctgaactacaagtacccagccctgaacgtgaccatgcccaacaacgacaacttcgacaagctgtacatctggggcgtgcaccacccatccaccgacaaggaccagacctccctgtacatccaggccagcggaagggtgaccgtgtccaccaagaggagccagcaggccgtgatcccaaacatcggatccaggccacgggtgagggacatcccctcccggatcagcatctactggaccatcgtgaggccaggcgacatcctgctgatcaacagcaacggcaacctgatcgcccccagaggctacttcaagatccgctccggcaagtccagcatcatgcggagcgacgcccccatcggcaactgcaacagcgagtgcatcaccccaaacggctccatcagcaacgacaagcccttccagaacgtgaacaagatcacctacggcgcctgcccaaggtacatcaagcagaacaccctgaagctggccaccggcatgagaaacatccccgagaagcagaccaggggaatcttcggagctaaggctggcttcatcgagaacggctgggagggcatggtgaacggctggtacggcttcagacaccagaactccgagggaaggggacaggctgctgacctgaagagcacccaggccgccatcgaccagatcaacggcaagctgaacagactgatcggcaagaccaacgagaagttccaccagatcgagaaggagttctccgagatcgagggccggatccaggacctggagaggtacgtggaggacaccaagatcgacatctggagctacaacgccgagctgctggtggccatggagaaccagcacaccatcgacctgaccgactccgagatgagcaagctgttcgagagaaccaggagacagctgcgcgagaacgccgaggacatgggcaacggctgcctgaagatctaccacaagtgcgacaactcctgcatggagagcatccggaacggcacctacgaccacgacatctaccggaacgaggccctgaacaacaggttccagatcaagggcgtggagctgaagagcgagtacaaggactggatcctgtggatctccttcgccaccagctgcttcctgctgtgcgccgtgctgctgggcttcatcatgtgggcctgccagaagggcaacatcaagtgcaacatctgcatc

SEQ ID NO: 122 - DNA, 1698 bp, synthetic construct
  misc_feature 1..1698: note = synthetically-generated coding sequence
  source 1..1698: mol_type = other DNA
atgaaggccatcatcgccttctcctgcatcctgtgccagatcttcgcccagaagctgcccggcaacgacaactccaccgccaccctgtgcctgggacaccacgccgtgagcaacggcaccctggtgaagaccatcaccgacgaccaggtggaggtgaccaacgccaccgagctggtgcagaacttctccatgggcaagatctgcaagaacccccacaggatcctggacggcgccaactgcaccctgatcgacagcctgctgggcgacccacactgcgacggcttccagaacgagaagtgggacctgttcatcgagaggtccaaggccttcagcaactgctacccctacgacgtgccagactacgcctccctgagaagcctgatcgcctccagcggcaccctggagttcaacaacgagtccttcaactggaccggagtgacccagaacggaggatccagcgcctgcaagaggggacccaacaactccttcttcagcagactgaactggctgacccacctgaacttcaagtaccccgccctggaggtgaccatgccaaacaacgagcagttcgacaagctgtacatctggggagtgcaccacccagctaccgacaaggaccagatcagcctgtacgctcaggctgctggaaggatcatcgtgtccaccaagagaagccagcagaccatcatccccaacatcggctccaggccatggatcagaggcgtgtccagcatcatcagcatccactggaccatcgtgaagcccggcgacatgctgctgatcaactccaccggcaacatcatcgccccacgcggctacttcaagatccagaccggcaagtccagcgtgatgcggagcgacgctccaatcggcaagtgcaactccgcctgcatcaccccaaacggaagcatccccaacgaccgcccattccagaacgtgaacaagatcacctacggcgcctgccccaagtacgtgaagcagaacaccctgaagctggccaccggcatgaggaacatcccagagaggcagaccaggggaatcttcggagctatcgccggcttcatcgagaacggctgggagggcatgatcgacggctggtacggcttccgccaccacaactccgagggcaccggacaggctgctgacatcaagagcacccaggctgccatcaaccagatcaacggcaagctgaaccgcgtgatcgagaagaccaacgagaagttccaccagatcgagaaggagttcctggaggtggagggccggatccaggacatcgagaagtacatcgaggacaccaagatcgacctgtggtcctacaacgccgagctgctgatcgccctggagaaccagcacaccatcgacctggccgacagcgagatgaacaagctgttcgagaagaccaagaagcagctgagggagaacgccgaggacatcggcaacggctgcttcaagatctaccacaagtgcgacaacacctgcatcggcagcatcagaaacggcacctacaaccacgacgtgtaccgcgacgaggccgtgaacaaccggttccagatcaagggcgtgcagctgaagctgggctacaaggactggatcctgtggatctccttcgccatgagctgcttcctgctgtgcgtggccctgctgggcttcatcatgtgggcttgccagaggggaaacatcaggtgcaacatctgcgtg